European Patent Specification EP 3 872 091 B1, published June 14, 2023. Title: ANTIBODIES AGAINST SARS-COV-2 AND METHODS OF USING THE SAME. Applicant: Vir Biotechnology, Inc. Humabs Biomed SA. Application EP. The sequence listing filed with the application follows.

SEQUENCE LISTING (267 sequences)

SEQ ID NO: 1 - protein, 123 aa, Artificial Sequence
  Synthetic sequence SARS-CoV-2 S300-v1 mAb VH
QVQLVQSGAEVKKPGASVKVSCKASGYTFTDYYIHWVRQAPGQGPEWLGWVNGYSGATRYAQKYQGRVTMTRDTSISTAYMQLSRLRPDDTAVYYCARDRPSHEWAMYFFDNWGQGTLVTVSS

SEQ ID NO: 2 - protein, 8 aa, Artificial Sequence
  Synthetic sequence SARS-CoV-2 S300-v1 mAb CDRH1
GYTFTDYY

SEQ ID NO: 3 - protein, 8 aa, Artificial Sequence
  Synthetic sequence SARS-CoV-2 S300-v1 mAb CDRH2
VNGYSGAT

SEQ ID NO: 4 - protein, 16 aa, Artificial Sequence
  Synthetic sequence SARS-CoV-2 S300-v1 mAb CDRH3
ARDRPSHEWAMYFFDN

SEQ ID NO: 5 - protein, 109 aa, Artificial Sequence
  Synthetic sequence SARS-CoV-2 S300-v1 mAb VL (VK)
QIVLTQSPGTLSLSPGERATLSCRASQSVPSSCLAWYQQKPGQAPRLLIYGASGRATGIPDRFSGSGSGTDFTLTIRRLEPEDFAVYYCQQYGSSPPLTFGGGTKVEIK

SEQ ID NO: 6 - protein, 7 aa, Artificial Sequence
  Synthetic sequence SARS-CoV-2 S300-v1 mAb CDRL1
QSVPSSC

SEQ ID NO: 7 - protein, 3 aa, Artificial Sequence
  Synthetic sequence SARS-CoV-2 S300-v1 mAb CDRL2
GAS

SEQ ID NO: 8 - protein, 10 aa, Artificial Sequence
  Synthetic sequence SARS-CoV-2 S300-v1 mAb CDRL3
QQYGSSPPLT

SEQ ID NO: 9 - protein, 123 aa, Artificial Sequence
  Synthetic sequence SARS-CoV-2 S300-v1.1 mAb VH
QVQLVQSGAEVKKPGASVKVSCKASGYTFTDYYIHWVRQAPGQGPEWLGWVQGYSGATRYAQKYQGRVTMTRDTSISTAYMQLSRLRPDDTAVYYCARDRPSHEWAMYFFDNWGQGTLVTVSS

SEQ ID NO: 10 - protein, 123 aa, Artificial Sequence
  Synthetic sequence SARS-CoV-2 S300-v1.2 mAb VH
QVQLVQSGAEVKKPGASVKVSCKASGYTFTDYYIHWVRQAPGQGPEWLGWVNAYSGATRYAQKYQGRVTMTRDTSISTAYMQLSRLRPDDTAVYYCARDRPSHEWAMYFFDNWGQGTLVTVSS

SEQ ID NO: 11 - protein, 123 aa, Artificial Sequence
  Synthetic sequence SARS-CoV-2 S300-v1.3 mAb VH
QVQLVQSGAEVKKPGASVKVSCKASGYTFTDYYIHWVRQAPGQGPEWLGWVNSYSGATRYAQKYQGRVTMTRDTSISTAYMQLSRLRPDDTAVYYCARDRPSHEWAMYFFDNWGQGTLVTVSS

SEQ ID NO: 12 - protein, 123 aa, Artificial Sequence
  Synthetic sequence SARS-CoV-2 S300-v1.4 mAb VH
QVQLVQSGAEVKKPGASVKVSCKASGYTFTDYYIHWVRQAPGQGPEWLGWVNPYSGATRYAQKYQGRVTMTRDTSISTAYMQLSRLRPDDTAVYYCARDRPSHEWAMYFFDNWGQGTLVTVSS

SEQ ID NO: 13 - protein, 123 aa, Artificial Sequence
  Synthetic sequence SARS-CoV-2 S300-v1.5 mAb VH
QVQLVQSGAEVKKPGASVKVSCKASGYTFTDYYIHWVRQAPGQGPEWLGWVNQYSGATRYAQKYQGRVTMTRDTSISTAYMQLSRLRPDDTAVYYCARDRPSHEWAMYFFDNWGQGTLVTVSS

SEQ ID NO: 14 - protein, 123 aa, Artificial Sequence
  Synthetic sequence SARS-CoV-2 S300-v1.6 mAb VH
QVQLVQSGAEVKKPGASVKVSCKASGYTFTDYYIHWVRQAPGQGPEWLGWVLGYSGATRYAQKYQGRVTMTRDTSISTAYMQLSRLRPDDTAVYYCARDRPSHEWAMYFFDNWGQGTLVTVSS

SEQ ID NO: 15 - protein, 123 aa, Artificial Sequence
  Synthetic sequence SARS-CoV-2 S300-v1.7 mAb VH
QVQLVQSGAEVKKPGASVKVSCKASGYTFTDYYIHWVRQAPGQGPEWLGWVTGYSGATRYAQKYQGRVTMTRDTSISTAYMQLSRLRPDDTAVYYCARDRPSHEWAMYFFDNWGQGTLVTVSS

SEQ ID NO: 16 - protein, 8 aa, Artificial Sequence
  Synthetic sequence SARS-CoV-2 S300-v1.1 mAb CDRH2
VQGYSGAT

SEQ ID NO: 17 - protein, 8 aa, Artificial Sequence
  Synthetic sequence SARS-CoV-2 S300-v1.2 mAb CDRH2
VNAYSGAT

SEQ ID NO: 18 - protein, 8 aa, Artificial Sequence
  Synthetic sequence SARS-CoV-2 S300-v1.3 mAb CDRH2
VNSYSGAT

SEQ ID NO: 19 - protein, 8 aa, Artificial Sequence
  Synthetic sequence SARS-CoV-2 S300-v1.4 mAb CDRH2
VNPYSGAT

SEQ ID NO: 20 - protein, 8 aa, Artificial Sequence
  Synthetic sequence SARS-CoV-2 S300-v1.5 mAb CDRH2
VNQYSGAT

SEQ ID NO: 21 - protein, 8 aa, Artificial Sequence
  Synthetic sequence SARS-CoV-2 S300-v1.6 mAb CDRH2
VLGYSGAT

SEQ ID NO: 22 - protein, 8 aa, Artificial Sequence
  Synthetic sequence SARS-CoV-2 S300-v1.7 mAb CDRH2
VTGYSGAT

SEQ ID NO: 23 - protein, 123 aa, Artificial Sequence
  Synthetic sequence SARS-CoV-2 S300-v1.8 mAb VH
QVQLVQSGAEVKKPGASVKVSCKASGYTFTDYYIHWVRQAPGQGPEWLGWVNGYSGATRYAQKYQGRVTMTRDTSISTAYMQLSRLRPDDTAVYYCARDRPSHEFAMYFFDNWGQGTLVTVSS

SEQ ID NO: 24 - protein, 123 aa, Artificial Sequence
  Synthetic sequence SARS-CoV-2 S300-v1.9 mAb VH
QVQLVQSGAEVKKPGASVKVSCKASGYTFTDYYIHWVRQAPGQGPEWLGWVNGYSGATRYAQKYQGRVTMTRDTSISTAYMQLSRLRPDDTAVYYCARDRPSHEYAMYFFDNWGQGTLVTVSS

SEQ ID NO: 25 - protein, 16 aa, Artificial Sequence
  Synthetic sequence SARS-CoV-2 S300-v1.8 mAb CDRH3
ARDRPSHEFAMYFFDN

SEQ ID NO: 26 - protein, 16 aa, Artificial Sequence
  Synthetic sequence SARS-CoV-2 S300-v1.9 mAb CDRH3
ARDRPSHEYAMYFFDN

SEQ ID NO: 27 - protein, 123 aa, Artificial Sequence
  Synthetic sequence SARS-CoV-2 S300-v2 mAb VH
QVQLVQSGAEVKKPGASVKVSCKASGYTFTDYYIHWVRQAPGQGPEWLGFVNGYSGATRYAQKYQGRVTMTRDTSISTAYMQLSRLRPDDTAVYYCARDRPSHEWAMYFFDNWGQGTLVTVSS

SEQ ID NO: 28 - protein, 123 aa, Artificial Sequence
  Synthetic sequence SARS-CoV-2 S300-v2.1 mAb VH
QVQLVQSGAEVKKPGASVKVSCKASGYTFTDYYIHWVRQAPGQGPEWLGFVQGYSGATRYAQKYQGRVTMTRDTSISTAYMQLSRLRPDDTAVYYCARDRPSHEWAMYFFDNWGQGTLVTVSS

SEQ ID NO: 29 - protein, 123 aa, Artificial Sequence
  Synthetic sequence SARS-CoV-2 S300-v2.2 mAb VH
QVQLVQSGAEVKKPGASVKVSCKASGYTFTDYYIHWVRQAPGQGPEWLGFVNAYSGATRYAQKYQGRVTMTRDTSISTAYMQLSRLRPDDTAVYYCARDRPSHEWAMYFFDNWGQGTLVTVSS

SEQ ID NO: 30 - protein, 123 aa, Artificial Sequence
  Synthetic sequence SARS-CoV-2 S300-v2.3 mAb VH
QVQLVQSGAEVKKPGASVKVSCKASGYTFTDYYIHWVRQAPGQGPEWLGFVNSYSGATRYAQKYQGRVTMTRDTSISTAYMQLSRLRPDDTAVYYCARDRPSHEWAMYFFDNWGQGTLVTVSS

SEQ ID NO: 31 - protein, 123 aa, Artificial Sequence
  Synthetic sequence SARS-CoV-2 S300-v2.4 mAb VH
QVQLVQSGAEVKKPGASVKVSCKASGYTFTDYYIHWVRQAPGQGPEWLGFVNPYSGATRYAQKYQGRVTMTRDTSISTAYMQLSRLRPDDTAVYYCARDRPSHEWAMYFFDNWGQGTLVTVSS

SEQ ID NO: 32 - protein, 123 aa, Artificial Sequence
  Synthetic sequence SARS-CoV-2 S300-v2.5 mAb VH
QVQLVQSGAEVKKPGASVKVSCKASGYTFTDYYIHWVRQAPGQGPEWLGFVNQYSGATRYAQKYQGRVTMTRDTSISTAYMQLSRLRPDDTAVYYCARDRPSHEWAMYFFDNWGQGTLVTVSS

SEQ ID NO: 33 - protein, 123 aa, Artificial Sequence
  Synthetic sequence SARS-CoV-2 S300-v2.6 mAb VH
QVQLVQSGAEVKKPGASVKVSCKASGYTFTDYYIHWVRQAPGQGPEWLGFVLGYSGATRYAQKYQGRVTMTRDTSISTAYMQLSRLRPDDTAVYYCARDRPSHEWAMYFFDNWGQGTLVTVSS

SEQ ID NO: 34 - protein, 123 aa, Artificial Sequence
  Synthetic sequence SARS-CoV-2 S300-v2.7 mAb VH
QVQLVQSGAEVKKPGASVKVSCKASGYTFTDYYIHWVRQAPGQGPEWLGFVTGYSGATRYAQKYQGRVTMTRDTSISTAYMQLSRLRPDDTAVYYCARDRPSHEWAMYFFDNWGQGTLVTVSS

SEQ ID NO: 35 - protein, 123 aa, Artificial Sequence
  Synthetic sequence SARS-CoV-2 S300-v2.8 mAb VH
QVQLVQSGAEVKKPGASVKVSCKASGYTFTDYYIHWVRQAPGQGPEWLGFVNGYSGATRYAQKYQGRVTMTRDTSISTAYMQLSRLRPDDTAVYYCARDRPSHEFAMYFFDNWGQGTLVTVSS

SEQ ID NO: 36 - protein, 123 aa, Artificial Sequence
  Synthetic sequence SARS-CoV-2 S300-v2.9 mAb VH
QVQLVQSGAEVKKPGASVKVSCKASGYTFTDYYIHWVRQAPGQGPEWLGFVNGYSGATRYAQKYQGRVTMTRDTSISTAYMQLSRLRPDDTAVYYCARDRPSHEYAMYFFDNWGQGTLVTVSS

SEQ ID NO: 37 - protein, 123 aa, Artificial Sequence
  Synthetic sequence SARS-CoV-2 S300-v3 mAb VH
QVQLVQSGAEVKKPGASVKVSCKASGYTFTDYYIHWVRQAPGQGPEWLGYVNGYSGATRYAQKYQGRVTMTRDTSISTAYMQLSRLRPDDTAVYYCARDRPSHEWAMYFFDNWGQGTLVTVSS

SEQ ID NO: 38 - protein, 123 aa, Artificial Sequence
  Synthetic sequence SARS-CoV-2 S300-v3.1 mAb VH
QVQLVQSGAEVKKPGASVKVSCKASGYTFTDYYIHWVRQAPGQGPEWLGYVQGYSGATRYAQKYQGRVTMTRDTSISTAYMQLSRLRPDDTAVYYCARDRPSHEWAMYFFDNWGQGTLVTVSS

SEQ ID NO: 39 - protein, 123 aa, Artificial Sequence
  Synthetic sequence SARS-CoV-2 S300-v3.2 mAb VH
QVQLVQSGAEVKKPGASVKVSCKASGYTFTDYYIHWVRQAPGQGPEWLGYVNAYSGATRYAQKYQGRVTMTRDTSISTAYMQLSRLRPDDTAVYYCARDRPSHEWAMYFFDNWGQGTLVTVSS

SEQ ID NO: 40 - protein, 123 aa, Artificial Sequence
  Synthetic sequence SARS-CoV-2 S300-v3.3 mAb VH
QVQLVQSGAEVKKPGASVKVSCKASGYTFTDYYIHWVRQAPGQGPEWLGYVNSYSGATRYAQKYQGRVTMTRDTSISTAYMQLSRLRPDDTAVYYCARDRPSHEWAMYFFDNWGQGTLVTVSS

SEQ ID NO: 41 - protein, 123 aa, Artificial Sequence
  Synthetic sequence SARS-CoV-2 S300-v3.4 mAb VH
QVQLVQSGAEVKKPGASVKVSCKASGYTFTDYYIHWVRQAPGQGPEWLGYVNPYSGATRYAQKYQGRVTMTRDTSISTAYMQLSRLRPDDTAVYYCARDRPSHEWAMYFFDNWGQGTLVTVSS

SEQ ID NO: 42 - protein, 123 aa, Artificial Sequence
  Synthetic sequence SARS-CoV-2 S300-v3.5 mAb VH
QVQLVQSGAEVKKPGASVKVSCKASGYTFTDYYIHWVRQAPGQGPEWLGYVNQYSGATRYAQKYQGRVTMTRDTSISTAYMQLSRLRPDDTAVYYCARDRPSHEWAMYFFDNWGQGTLVTVSS

SEQ ID NO: 43 - protein, 123 aa, Artificial Sequence
  Synthetic sequence SARS-CoV-2 S300-v3.6 mAb VH
QVQLVQSGAEVKKPGASVKVSCKASGYTFTDYYIHWVRQAPGQGPEWLGYVLGYSGATRYAQKYQGRVTMTRDTSISTAYMQLSRLRPDDTAVYYCARDRPSHEWAMYFFDNWGQGTLVTVSS

SEQ ID NO: 44 - protein, 123 aa, Artificial Sequence
  Synthetic sequence SARS-CoV-2 S300-v3.7 mAb VH
QVQLVQSGAEVKKPGASVKVSCKASGYTFTDYYIHWVRQAPGQGPEWLGYVTGYSGATRYAQKYQGRVTMTRDTSISTAYMQLSRLRPDDTAVYYCARDRPSHEWAMYFFDNWGQGTLVTVSS

SEQ ID NO: 45 - protein, 123 aa, Artificial Sequence
  Synthetic sequence SARS-CoV-2 S300-v3.8 mAb VH
QVQLVQSGAEVKKPGASVKVSCKASGYTFTDYYIHWVRQAPGQGPEWLGYVNGYSGATRYAQKYQGRVTMTRDTSISTAYMQLSRLRPDDTAVYYCARDRPSHEFAMYFFDNWGQGTLVTVSS

SEQ ID NO: 46 - protein, 123 aa, Artificial Sequence
  Synthetic sequence SARS-CoV-2 S300-v3.9 mAb VH
QVQLVQSGAEVKKPGASVKVSCKASGYTFTDYYIHWVRQAPGQGPEWLGYVNGYSGATRYAQKYQGRVTMTRDTSISTAYMQLSRLRPDDTAVYYCARDRPSHEYAMYFFDNWGQGTLVTVSS

SEQ ID NO: 47 - protein, 109 aa, Artificial Sequence
  Synthetic sequence SARS-CoV-2 S300-v10 mAb VL (VK)
QIVLTQSPGTLSLSPGERATLSCRASQSVPSSYLAWYQQKPGQAPRLLIYGASGRATGIPDRFSGSGSGTDFTLTIRRLEPEDFAVYYCQQYGSSPPLTFGGGTKVEIK

SEQ ID NO: 48 - protein, 109 aa, Artificial Sequence
  Synthetic sequence SARS-CoV-2 S300-v11 mAb VL (VK)
QIVLTQSPGTLSLSPGERATLSCRASQSVPSSSLAWYQQKPGQAPRLLIYGASGRATGIPDRFSGSGSGTDFTLTIRRLEPEDFAVYYCQQYGSSPPLTFGGGTKVEIK

SEQ ID NO: 49 - protein, 109 aa, Artificial Sequence
  Synthetic sequence SARS-CoV-2 S300-v12 mAb VL (VK)
QIVLTQSPGTLSLSPGERATLSCRASQSVPSSTLAWYQQKPGQAPRLLIYGASGRATGIPDRFSGSGSGTDFTLTIRRLEPEDFAVYYCQQYGSSPPLTFGGGTKVEIK

SEQ ID NO: 50 - protein, 109 aa, Artificial Sequence
  Synthetic sequence SARS-CoV-2 S300-v13 mAb VL (VK)
QIVLTQSPGTLSLSPGERATLSCRASQSVPSSALAWYQQKPGQAPRLLIYGASGRATGIPDRFSGSGSGTDFTLTIRRLEPEDFAVYYCQQYGSSPPLTFGGGTKVEIK

SEQ ID NO: 51 - protein, 7 aa, Artificial Sequence
  Synthetic sequence SARS-CoV-2 S300-v10 mAb CDRL1
QSVPSSY

SEQ ID NO: 52 - protein, 7 aa, Artificial Sequence
  Synthetic sequence SARS-CoV-2 S300-v11 mAb CDRL1
QSVPSSS

SEQ ID NO: 53 - protein, 7 aa, Artificial Sequence
  Synthetic sequence SARS-CoV-2 S300-v12 mAb CDRL1
QSVPSST

SEQ ID NO: 54 - protein, 7 aa, Artificial Sequence
  Synthetic sequence SARS-CoV-2 S300-v13 mAb CDRL1
QSVPSSA

SEQ ID NO: 55 - protein, 121 aa, Artificial Sequence
  Synthetic sequence SARS-CoV-2 S302 mAb VH
QVQLVESGGGVVQPGRSLRLSCAASGFTFSSYGMHWVRQAPGKGLEWVAVISYDGSNKYYADSVKGRFTISRDNSKNTLYLQMNSLRAEDTAVYYCAKDISSGWDRVFDYWGQGTLVTVSS

SEQ ID NO: 56 - protein, 8 aa, Artificial Sequence
  Synthetic sequence SARS-CoV-2 S302 mAb CDRH1
GFTFSSYG

SEQ ID NO: 57 - protein, 8 aa, Artificial Sequence
  Synthetic sequence SARS-CoV-2 S302 mAb CDRH2
ISYDGSNK

SEQ ID NO: 58 - protein, 14 aa, Artificial Sequence
  Synthetic sequence SARS-CoV-2 S302 mAb CDRH3
AKDISSGWDRVFDY

SEQ ID NO: 59 - protein, 108 aa, Artificial Sequence
  Synthetic sequence SARS-CoV-2 S302 mAb VL (VK)
EILLTQSPGTLSLSPGERATLSCRTSQSVGSSYLAWYQQKPGQAPRLLIYAASSRAIGIPDRFSGSGSGTDFTLTISRLEPEDFAVYYCQQYGSSPWTFGQGTKVEIK

SEQ ID NO: 60 - protein, 7 aa, Artificial Sequence
  Synthetic sequence SARS-CoV-2 S302 mAb CDRL1
QSVGSSY

SEQ ID NO: 61 - protein, 3 aa, Artificial Sequence
  Synthetic sequence SARS-CoV-2 S302 mAb CDRL2
AAS

SEQ ID NO: 62 - protein, 9 aa, Artificial Sequence
  Synthetic sequence SARS-CoV-2 S302 mAb CDRL3
QQYGSSPWT

SEQ ID NO: 63 - protein, 124 aa, Artificial Sequence
  Synthetic sequence SARS-CoV-2 S303-v1 mAb VH
EVQLVESGGGLVKPGGSLRLSCAASGFTFLTYSMNWVRQTPGKRLQWVSAISGSGGATYYADSVKGRFTISRDNSKNTLYLQMNTVTADDTAIYFCARERDDIFPMGLNAFDIWGQGAMVIVSS

SEQ ID NO: 64 - protein, 8 aa, Artificial Sequence
  Synthetic sequence SARS-CoV-2 S303-v1 mAb CDRH1
GFTFLTYS

SEQ ID NO: 65 - protein, 8 aa, Artificial Sequence
  Synthetic sequence SARS-CoV-2 S303-v1 mAb CDRH2
ISGSGGAT

SEQ ID NO: 66 - protein, 17 aa, Artificial Sequence
  Synthetic sequence SARS-CoV-2 S303-v1 mAb CDRH3
ARERDDIFPMGLNAFDI

SEQ ID NO: 67 - protein, 107 aa, Artificial Sequence
  Synthetic sequence SARS-CoV-2 S303-v1 mAb VL (VK)
DIQMTQSPSTLSASVGDRVTITCRASQSISNWLAWYQQKPGKAPKLLIYKASSLESGVPSRFSGSGSGTEFTLTISSLQPDDSATYYCQQYDTYSWTFGQGTKVEIK

SEQ ID NO: 68 - protein, 6 aa, Artificial Sequence
  Synthetic sequence SARS-CoV-2 S303-v1 mAb CDRL1
QSISNW

SEQ ID NO: 69 - protein, 3 aa, Artificial Sequence
  Synthetic sequence SARS-CoV-2 S303-v1 mAb CDRL2
KAS

SEQ ID NO: 70 - protein, 9 aa, Artificial Sequence
  Synthetic sequence SARS-CoV-2 S303-v1 mAb CDRL3
QQYDTYSWT

SEQ ID NO: 71 - protein, 107 aa, Artificial Sequence
  Synthetic sequence SARS-CoV-2 S303-v2 mAb VL (VK)
DIQMTQSPSTLSASVGDRVTITCRASQSISNFLAWYQQKPGKAPKLLIYKASSLESGVPSRFSGSGSGTEFTLTISSLQPDDSATYYCQQYDTYSWTFGQGTKVEIK

SEQ ID NO: 72 - protein, 107 aa, Artificial Sequence
  Synthetic sequence SARS-CoV-2 S303-v3 mAb VL (VK)
DIQMTQSPSTLSASVGDRVTITCRASQSISNYLAWYQQKPGKAPKLLIYKASSLESGVPSRFSGSGSGTEFTLTISSLQPDDSATYYCQQYDTYSWTFGQGTKVEIK

SEQ ID NO: 73 - protein, 6 aa, Artificial Sequence
  Synthetic sequence SARS-CoV-2 S303-v2 mAb CDRL1
QSISNF

SEQ ID NO: 74 - protein, 6 aa, Artificial Sequence
  Synthetic sequence SARS-CoV-2 S303-v3 mAb CDRL1
QSISNY

SEQ ID NO: 75 - protein, 107 aa, Artificial Sequence
  Synthetic sequence SARS-CoV-2 S303-v4 mAb VL (VK)
DIQMTQSPSTLSASVGDRVTITCRASQSISNWLAWYQQKPGKAPKLLIYKASSLESGVPSRFSGSGSGTEFTLTISSLQPDDSATYYCQQYDTYSFTFGQGTKVEIK

SEQ ID NO: 76 - protein, 107 aa, Artificial Sequence
  Synthetic sequence SARS-CoV-2 S303-v5 mAb VL (VK)
DIQMTQSPSTLSASVGDRVTITCRASQSISNWLAWYQQKPGKAPKLLIYKASSLESGVPSRFSGSGSGTEFTLTISSLQPDDSATYYCQQYDTYSYTFGQGTKVEIK

SEQ ID NO: 77 - protein, 9 aa, Artificial Sequence
  Synthetic sequence SARS-CoV-2 S303-v4 mAb CDRL3
QQYDTYSFT

SEQ ID NO: 78 - protein, 9 aa, Artificial Sequence
  Synthetic sequence SARS-CoV-2 S303-v5 mAb CDRL3
QQYDTYSYT

SEQ ID NO: 79 - protein, 120 aa, Artificial Sequence
  Synthetic sequence SARS-CoV-2 S304 mAb VH
EVQLVESGGGLVQPGGSLRLSCAASGFTFSSYDMHWVRQTTGKGLEWVSTIGTAGDTYYPDSVKGRFTISREDAKNSLYLQMNSLRAGDTAVYYCARGDSSGYYYYFDYWGQGTLLTVSS

SEQ ID NO: 80 - protein, 8 aa, Artificial Sequence
  Synthetic sequence SARS-CoV-2 S304 mAb CDRH1
GFTFSSYD

SEQ ID NO: 81 - protein, 7 aa, Artificial Sequence
  Synthetic sequence SARS-CoV-2 S304 mAb CDRH2
IGTAGDT

SEQ ID NO: 82 - protein, 14 aa, Artificial Sequence
  Synthetic sequence SARS-CoV-2 S304 mAb CDRH3
ARGDSSGYYYYFDY

SEQ ID NO: 83 - protein, 108 aa, Artificial Sequence
  Synthetic sequence SARS-CoV-2 S304 mAb VL (VK)
DIQMTQSPSSLSAAVGDRVTITCRASQSIGSYLNWYQQKPGKAPKLLIYAASSLQSGVPSRFSGSGSGTDFTLTISSLQPEDFAIYYCQQSYVSPTYTFGPGTKVDIK

SEQ ID NO: 84 - protein, 6 aa, Artificial Sequence
  Synthetic sequence SARS-CoV-2 S304 mAb CDRL1
QSIGSY

SEQ ID NO: 85 - protein, 3 aa, Artificial Sequence
  Synthetic sequence SARS-CoV-2 S304 mAb CDRL2
AAS

SEQ ID NO: 86 - protein, 10 aa, Artificial Sequence
  Synthetic sequence SARS-CoV-2 S304 mAb CDRL3
QQSYVSPTYT

SEQ ID NO: 87 - protein, 123 aa, Artificial Sequence
  Synthetic sequence SARS-CoV-2 S306 mAb VH
QVQLVQSGAEVKKPGASVKVSCKASTYTFTSFGISWVRQAPGQGLEWMGWITTYSGDTNYAQKFQGRVTMTTDTSTNTAYMELRSLRSDDTAVYYCASDYFDSSGYYHSFDYWGQGTLVTVSS

SEQ ID NO: 88 - protein, 8 aa, Artificial Sequence
  Synthetic sequence SARS-CoV-2 S306 mAb CDRH1
TYTFTSFG

SEQ ID NO: 89 - protein, 8 aa, Artificial Sequence
  Synthetic sequence SARS-CoV-2 S306 mAb CDRH2
ITTYSGDT

SEQ ID NO: 90 - protein, 16 aa, Artificial Sequence
  Synthetic sequence SARS-CoV-2 S306 mAb CDRH3
ASDYFDSSGYYHSFDY

SEQ ID NO: 91 - protein, 109 aa, Artificial Sequence
  Synthetic sequence SARS-CoV-2 S306 mAb VL (VK)
EIVLTQSPDTLSLSPGERATLSCRASQSVSSYLAWYQQRPGQAPRLLIYDASKRATGIPARFSGSGSGTDFTLTISSLEPEDFAVYYCQQRSNWPPGCSFGQGTKVEIK

SEQ ID NO: 92 - protein, 6 aa, Artificial Sequence
  Synthetic sequence SARS-CoV-2 S306 mAb CDRL1
QSVSSY

SEQ ID NO: 93 - protein, 3 aa, Artificial Sequence
  Synthetic sequence SARS-CoV-2 S306 mAb CDRL2
DAS

SEQ ID NO: 94 - protein, 11 aa, Artificial Sequence
  Synthetic sequence SARS-CoV-2 S306 mAb CDRL3
QQRSNWPPGCS

SEQ ID NO: 95 - protein, 127 aa, Artificial Sequence
  Synthetic sequence SARS-CoV-2 S308-v1 mAb VH
QVQLVESGGGVVQPGRSLRLSCAASRFTFSSYGMHWVRQAPGKGLEWVAVIWHDGNNKHYGDSVKGRVTISRDNSKNTLYLQMTSLRAEDTAVYYCARAVTTFKGSGRARMRGMDVWGQGTTVTVSS

SEQ ID NO: 96 - protein, 8 aa, Artificial Sequence
  Synthetic sequence SARS-CoV-2 S308-v1 mAb CDRH1
RFTFSSYG

SEQ ID NO: 97 - protein, 8 aa, Artificial Sequence
  Synthetic sequence SARS-CoV-2 S308-v1 mAb CDRH2
IWHDGNNK

SEQ ID NO: 98 - protein, 20 aa, Artificial Sequence
  Synthetic sequence SARS-CoV-2 S308-v1 mAb CDRH3
ARAVTTFKGSGRARMRGMDV

SEQ ID NO: 99 - protein, 107 aa, Artificial Sequence
  Synthetic sequence SARS-CoV-2 S308-v1 mAb VL (VK)
DIQLTQSPSFLSASVGDRVTITCRASQGINTYLAWYQQKPGKAPKLLIYAASTLQSGVPSRFSGSGSGTEFTLTISSLQPEDFATYYCQHLDTYPFTFGPGTKVDIK

SEQ ID NO: 100 - protein, 6 aa, Artificial Sequence
  Synthetic sequence SARS-CoV-2 S308-v1 mAb CDRL1
QGINTY

SEQ ID NO: 101 - protein, 3 aa, Artificial Sequence
  Synthetic sequence SARS-CoV-2 S308-v1 mAb CDRL2
AAS

SEQ ID NO: 102 - protein, 9 aa, Artificial Sequence
  Synthetic sequence SARS-CoV-2 S308-v1 mAb CDRL3
QHLDTYPFT

SEQ ID NO: 103 - protein, 127 aa, Artificial Sequence
  Synthetic sequence SARS-CoV-2 S308-v2 mAb VH
QVQLVESGGGVVQPGRSLRLSCAASRFTFSSYGMHWVRQAPGKGLEWVAVIWHDGNNKHYGDSVKGRVTISRDNSKNTLYLQMTSLRAEDTAVYYCARAVTTFKGSGRARLRGMDVWGQGTTVTVSS

SEQ ID NO: 104 - protein, 20 aa, Artificial Sequence
  Synthetic sequence SARS-CoV-2 S308-v2 mAb CDRH3
ARAVTTFKGSGRARLRGMDV

SEQ ID NO: 105 - protein, 127 aa, Artificial Sequence [sequence omitted]

SEQ ID NO: 106 - protein, 8 aa, Artificial Sequence
  Synthetic sequence SARS-CoV-2 S309-v1 mAb CDRH1
GYPFTSYG

SEQ ID NO: 107 - protein, 8 aa, Artificial Sequence
  Synthetic sequence SARS-CoV-2 S309-v1 mAb CDRH2
ISTYNGNT

SEQ ID NO: 108 - protein, 20 aa, Artificial Sequence
  Synthetic sequence SARS-CoV-2 S309-v1 mAb CDRH3
ARDYTRGAWFGESLIGGFDN

SEQ ID NO: 109 - protein, 107 aa, Artificial Sequence
  Synthetic sequence SARS-CoV-2 S309-v1 mAb VL (VK)
DIQMTQSPSSLSTSVGDRVTITCRASQGINNYVAWYQQKPGKVPKLLIYGASTLQSGVPSRFRGSGSGTGFTLTISSLQPEDVASYYCRKYNSAPWTFGQGTRVEIK

SEQ ID NO: 110 - protein, 6 aa, Artificial Sequence
  Synthetic sequence SARS-CoV-2 S309-v1 mAb CDRL1
QGINNY

SEQ ID NO: 111 - protein, 3 aa, Artificial Sequence
  Synthetic sequence SARS-CoV-2 S309-v1 mAb CDRL2
GAS

SEQ ID NO: 112 - protein, 9 aa, Artificial Sequence
  Synthetic sequence SARS-CoV-2 S309-v1 mAb CDRL3
RKYNSAPWT

SEQ ID NO: 113 - protein, 127 aa, Artificial Sequence
  Synthetic sequence SARS-CoV-2 S309-v1.1 mAb VH
QVQLVQSGAEVKKPGASVKVSCKASGYPFTSYGISWVRQAPGQGLEWMGWISTYQGNTNYAQKFQGRVTMTTDTSTTTGYMELRRLRSDDTAVYYCARDYTRGAWFGESLIGGFDNWGQGTLVTVSS

SEQ ID NO: 114 - protein, 127 aa, Artificial Sequence
  Synthetic sequence SARS-CoV-2 S309-v1.2 mAb VH
QVQLVQSGAEVKKPGASVKVSCKASGYPFTSYGISWVRQAPGQGLEWMGWISTYNSNTNYAQKFQGRVTMTTDTSTTTGYMELRRLRSDDTAVYYCARDYTRGAWFGESLIGGFDNWGQGTLVTVSS

SEQ ID NO: 115 - protein, 127 aa, Artificial Sequence
  Synthetic sequence SARS-CoV-2 S309-v1.3 mAb VH
QVQLVQSGAEVKKPGASVKVSCKASGYPFTSYGISWVRQAPGQGLEWMGWISTYNANTNYAQKFQGRVTMTTDTSTTTGYMELRRLRSDDTAVYYCARDYTRGAWFGESLIGGFDNWGQGTLVTVSS

SEQ ID NO: 116 - protein, 127 aa, Artificial Sequence
  Synthetic sequence SARS-CoV-2 S309-v1.4 mAb VH
QVQLVQSGAEVKKPGASVKVSCKASGYPFTSYGISWVRQAPGQGLEWMGWISTYNQNTNYAQKFQGRVTMTTDTSTTTGYMELRRLRSDDTAVYYCARDYTRGAWFGESLIGGFDNWGQGTLVTVSS

SEQ ID NO: 117 - protein, 127 aa, Artificial Sequence
  Synthetic sequence SARS-CoV-2 S309-v1.5 mAb VH
QVQLVQSGAEVKKPGASVKVSCKASGYPFTSYGISWVRQAPGQGLEWMGWISTYLGNTNYAQKFQGRVTMTTDTSTTTGYMELRRLRSDDTAVYYCARDYTRGAWFGESLIGGFDNWGQGTLVTVSS

SEQ ID NO: 118 - protein, 127 aa, Artificial Sequence
  Synthetic sequence SARS-CoV-2 S309-v1.6 mAb VH
QVQLVQSGAEVKKPGASVKVSCKASGYPFTSYGISWVRQAPGQGLEWMGWISTYTGNTNYAQKFQGRVTMTTDTSTTTGYMELRRLRSDDTAVYYCARDYTRGAWFGESLIGGFDNWGQGTLVTVSS

SEQ ID NO: 119 - protein, 127 aa, Artificial Sequence
  Synthetic sequence SARS-CoV-2 S309-v1.7 mAb VH
QVQLVQSGAEVKKPGASVKVSCKASGYPFTSYGISWVRQAPGQGLEWMGWISTYNGNTNYAQKFQGRVTMTTDTSTTTGYMELRRLRSDDTAVYYCARDYTRGAFFGESLIGGFDNWGQGTLVTVSS

SEQ ID NO: 120 - protein, 127 aa, Artificial Sequence
  Synthetic sequence SARS-CoV-2 S309-v1.8 mAb VH
QVQLVQSGAEVKKPGASVKVSCKASGYPFTSYGISWVRQAPGQGLEWMGWISTYNGNTNYAQKFQGRVTMTTDTSTTTGYMELRRLRSDDTAVYYCARDYTRGAYFGESLIGGFDNWGQGTLVTVSS

SEQ ID NO: 121 - protein, 8 aa, Artificial Sequence
  Synthetic sequence SARS-CoV-2 S309-v1.1 mAb CDRH2
ISTYQGNT

SEQ ID NO: 122 - protein, 8 aa, Artificial Sequence
  Synthetic sequence SARS-CoV-2 S309-v1.2 mAb CDRH2
ISTYNSNT

SEQ ID NO: 123 - protein, 8 aa, Artificial Sequence
  Synthetic sequence SARS-CoV-2 S309-v1.3 mAb CDRH2
ISTYNANT

SEQ ID NO: 124 - protein, 8 aa, Artificial Sequence
  Synthetic sequence SARS-CoV-2 S309-v1.4 mAb CDRH2
ISTYNQNT

SEQ ID NO: 125 - protein, 8 aa, Artificial Sequence
  Synthetic sequence SARS-CoV-2 S309-v1.5 mAb CDRH2
ISTYLGNT

SEQ ID NO: 126 - protein, 8 aa, Artificial Sequence
  Synthetic sequence SARS-CoV-2 S309-v1.6 mAb CDRH2
ISTYTGNT

SEQ ID NO: 127 - protein, 20 aa, Artificial Sequence
  Synthetic sequence SARS-CoV-2 S309-v1.7 mAb CDRH3
ARDYTRGAFFGESLIGGFDN

SEQ ID NO: 128 - protein, 20 aa, Artificial Sequence
  Synthetic sequence SARS-CoV-2 S309-v1.8 mAb CDRH3
ARDYTRGAYFGESLIGGFDN

SEQ ID NO: 129 - protein, 127 aa, Artificial Sequence
  Synthetic sequence SARS-CoV-2 S309-v2 mAb VH
QVQLVQSGAEVKKPGASVKVSCKASGYPFTSYGISWVRQAPGQGLEWMGFISTYNGNTNYAQKFQGRVTMTTDTSTTTGYMELRRLRSDDTAVYYCARDYTRGAWFGESLIGGFDNWGQGTLVTVSS

SEQ ID NO: 130 - protein, 127 aa, Artificial Sequence
  Synthetic sequence SARS-CoV-2 S309-v2.1 mAb VH
QVQLVQSGAEVKKPGASVKVSCKASGYPFTSYGISWVRQAPGQGLEWMGFISTYQGNTNYAQKFQGRVTMTTDTSTTTGYMELRRLRSDDTAVYYCARDYTRGAWFGESLIGGFDNWGQGTLVTVSS

SEQ ID NO: 131 - protein, 127 aa, Artificial Sequence
  Synthetic sequence SARS-CoV-2 S309-v2.2 mAb VH
QVQLVQSGAEVKKPGASVKVSCKASGYPFTSYGISWVRQAPGQGLEWMGFISTYNSNTNYAQKFQGRVTMTTDTSTTTGYMELRRLRSDDTAVYYCARDYTRGAWFGESLIGGFDNWGQGTLVTVSS

SEQ ID NO: 132 - protein, 127 aa, Artificial Sequence
  Synthetic sequence SARS-CoV-2 S309-v2.3 mAb VH
QVQLVQSGAEVKKPGASVKVSCKASGYPFTSYGISWVRQAPGQGLEWMGFISTYNANTNYAQKFQGRVTMTTDTSTTTGYMELRRLRSDDTAVYYCARDYTRGAWFGESLIGGFDNWGQGTLVTVSS

SEQ ID NO: 133 - protein, 127 aa, Artificial Sequence
  Synthetic sequence SARS-CoV-2 S309-v2.4 mAb VH
QVQLVQSGAEVKKPGASVKVSCKASGYPFTSYGISWVRQAPGQGLEWMGFISTYNQNTNYAQKFQGRVTMTTDTSTTTGYMELRRLRSDDTAVYYCARDYTRGAWFGESLIGGFDNWGQGTLVTVSS

SEQ ID NO: 134 - protein, 127 aa, Artificial Sequence
  Synthetic sequence SARS-CoV-2 S309-v2.5 mAb VH
QVQLVQSGAEVKKPGASVKVSCKASGYPFTSYGISWVRQAPGQGLEWMGFISTYLGNTNYAQKFQGRVTMTTDTSTTTGYMELRRLRSDDTAVYYCARDYTRGAWFGESLIGGFDNWGQGTLVTVSS

SEQ ID NO: 135 - protein, 127 aa, Artificial Sequence
  Synthetic sequence SARS-CoV-2 S309-v2.6 mAb VH
QVQLVQSGAEVKKPGASVKVSCKASGYPFTSYGISWVRQAPGQGLEWMGFISTYTGNTNYAQKFQGRVTMTTDTSTTTGYMELRRLRSDDTAVYYCARDYTRGAWFGESLIGGFDNWGQGTLVTVSS

SEQ ID NO: 136 - protein, 127 aa, Artificial Sequence
  Synthetic sequence SARS-CoV-2 S309-v2.7 mAb VH
QVQLVQSGAEVKKPGASVKVSCKASGYPFTSYGISWVRQAPGQGLEWMGFISTYNGNTNYAQKFQGRVTMTTDTSTTTGYMELRRLRSDDTAVYYCARDYTRGAFFGESLIGGFDNWGQGTLVTVSS

SEQ ID NO: 137 - protein, 127 aa, Artificial Sequence
  Synthetic sequence SARS-CoV-2 S309-v2.8 mAb VH
QVQLVQSGAEVKKPGASVKVSCKASGYPFTSYGISWVRQAPGQGLEWMGFISTYNGNTNYAQKFQGRVTMTTDTSTTTGYMELRRLRSDDTAVYYCARDYTRGAYFGESLIGGFDNWGQGTLVTVSS

SEQ ID NO: 138 - protein, 127 aa, Artificial Sequence
  Synthetic sequence SARS-CoV-2 S309-v3 mAb VH
QVQLVQSGAEVKKPGASVKVSCKASGYPFTSYGISWVRQAPGQGLEWMGYISTYNGNTNYAQKFQGRVTMTTDTSTTTGYMELRRLRSDDTAVYYCARDYTRGAWFGESLIGGFDNWGQGTLVTVSS

SEQ ID NO: 139 - protein, 127 aa, Artificial Sequence
  Synthetic sequence SARS-CoV-2 S309-v3.1 mAb VH
QVQLVQSGAEVKKPGASVKVSCKASGYPFTSYGISWVRQAPGQGLEWMGYISTYQGNTNYAQKFQGRVTMTTDTSTTTGYMELRRLRSDDTAVYYCARDYTRGAWFGESLIGGFDNWGQGTLVTVSS

SEQ ID NO: 140 - protein, 127 aa, Artificial Sequence
  Synthetic sequence SARS-CoV-2 S309-v3.2 mAb VH
QVQLVQSGAEVKKPGASVKVSCKASGYPFTSYGISWVRQAPGQGLEWMGYISTYNSNTNYAQKFQGRVTMTTDTSTTTGYMELRRLRSDDTAVYYCARDYTRGAWFGESLIGGFDNWGQGTLVTVSS

SEQ ID NO: 141 - protein, 127 aa, Artificial Sequence
  Synthetic sequence SARS-CoV-2 S309-v3.3 mAb VH
QVQLVQSGAEVKKPGASVKVSCKASGYPFTSYGISWVRQAPGQGLEWMGYISTYNANTNYAQKFQGRVTMTTDTSTTTGYMELRRLRSDDTAVYYCARDYTRGAWFGESLIGGFDNWGQGTLVTVSS

SEQ ID NO: 142 - protein, 127 aa, Artificial Sequence
  Synthetic sequence SARS-CoV-2 S309-v3.4 mAb VH
QVQLVQSGAEVKKPGASVKVSCKASGYPFTSYGISWVRQAPGQGLEWMGYISTYNQNTNYAQKFQGRVTMTTDTSTTTGYMELRRLRSDDTAVYYCARDYTRGAWFGESLIGGFDNWGQGTLVTVSS

SEQ ID NO: 143 - protein, 127 aa, Artificial Sequence
  Synthetic sequence SARS-CoV-2 S309-v3.5 mAb VH
QVQLVQSGAEVKKPGASVKVSCKASGYPFTSYGISWVRQAPGQGLEWMGYISTYLGNTNYAQKFQGRVTMTTDTSTTTGYMELRRLRSDDTAVYYCARDYTRGAWFGESLIGGFDNWGQGTLVTVSS

SEQ ID NO: 144 - protein, 127 aa, Artificial Sequence
  Synthetic sequence SARS-CoV-2 S309-v3.6 mAb VH
QVQLVQSGAEVKKPGASVKVSCKASGYPFTSYGISWVRQAPGQGLEWMGYISTYTGNTNYAQKFQGRVTMTTDTSTTTGYMELRRLRSDDTAVYYCARDYTRGAWFGESLIGGFDNWGQGTLVTVSS

SEQ ID NO: 145 - protein, 127 aa, Artificial Sequence
  Synthetic sequence SARS-CoV-2 S309-v3.7 mAb VH
QVQLVQSGAEVKKPGASVKVSCKASGYPFTSYGISWVRQAPGQGLEWMGYISTYNGNTNYAQKFQGRVTMTTDTSTTTGYMELRRLRSDDTAVYYCARDYTRGAFFGESLIGGFDNWGQGTLVTVSS

SEQ ID NO: 146 - protein, 127 aa, Artificial Sequence
  Synthetic sequence SARS-CoV-2 S309-v3.8 mAb VH
QVQLVQSGAEVKKPGASVKVSCKASGYPFTSYGISWVRQAPGQGLEWMGYISTYNGNTNYAQKFQGRVTMTTDTSTTTGYMELRRLRSDDTAVYYCARDYTRGAYFGESLIGGFDNWGQGTLVTVSS

SEQ ID NO: 147 - protein, 107 aa, Artificial Sequence
  Synthetic sequence SARS-CoV-2 S309-v9 mAb VL (VK)
DIQMTQSPSSLSTSVGDRVTITCRASQGINNYVAWYQQKPGKVPKLLIYGASTLQSGVPSRFRGSGSGTGFTLTISSLQPEDVASYYCRKYNSAPGTFGQGTRVEIK

SEQ ID NO: 148 - protein, 107 aa, Artificial Sequence
  Synthetic sequence SARS-CoV-2 S309-v10 mAb VL (VK)
DIQMTQSPSSLSTSVGDRVTITCRASQGINNYVAWYQQKPGKVPKLLIYGASTLQSGVPSRFRGSGSGTGFTLTISSLQPEDVASYYCRKYNSAPRTFGQGTRVEIK

SEQ ID NO: 149 - protein, 107 aa, Artificial Sequence
  Synthetic sequence SARS-CoV-2 S309-v11 mAb VL (VK)
DIQMTQSPSSLSTSVGDRVTITCRASQGINNYVAWYQQKPGKVPKLLIYGASTLQSGVPSRFRGSGSGTGFTLTISSLQPEDVASYYCRKYNSAPFTFGQGTRVEIK

SEQ ID NO: 150 - protein, 107 aa, Artificial Sequence
  Synthetic sequence SARS-CoV-2 S309-v12 mAb VL (VK)
DIQMTQSPSSLSTSVGDRVTITCRASQGINNYVAWYQQKPGKVPKLLIYGASTLQSGVPSRFRGSGSGTGFTLTISSLQPEDVASYYCRKYNSAPYTFGQGTRVEIK

SEQ ID NO: 151 - protein, 9 aa, Artificial Sequence
  Synthetic sequence SARS-CoV-2 S309-v9 mAb CDRL3
RKYNSAPGT

SEQ ID NO: 152 - protein, 9 aa, Artificial Sequence
  Synthetic sequence SARS-CoV-2 S309-v10 mAb CDRL3
RKYNSAPRT

SEQ ID NO: 153 - protein, 9 aa, Artificial Sequence
  Synthetic sequence SARS-CoV-2 S309-v11 mAb CDRL3
RKYNSAPFT

SEQ ID NO: 154 - protein, 9 aa, Artificial Sequence
  Synthetic sequence SARS-CoV-2 S309-v12 mAb CDRL3
RKYNSAPYT

SEQ ID NO: 155 - protein, 126 aa, Artificial Sequence
  Synthetic sequence SARS-CoV-2 S310 mAb VH
QVQLVQSGAELKKPGSSVKVSCKASGGTFNSYSFNWVRQAPGQGLEWLGGIIPVLGTSNYAQKFQGRVAVTADEFTTTAYMELSSLRSEDTAVYYCATRTYDSSGYRPYYYGLDVWGQGTPVTVSS

SEQ ID NO: 156 - protein, 8 aa, Artificial Sequence
  Synthetic sequence SARS-CoV-2 S310 mAb CDRH1
GGTFNSYS

SEQ ID NO: 157 - protein, 8 aa, Artificial Sequence
  Synthetic sequence SARS-CoV-2 S310 mAb CDRH2
IIPVLGTS

SEQ ID NO: 158 - protein, 19 aa, Artificial Sequence
  Synthetic sequence SARS-CoV-2 S310 mAb CDRH3
ATRTYDSSGYRPYYYGLDV

SEQ ID NO: 159 - protein, 110 aa, Artificial Sequence
  Synthetic sequence SARS-CoV-2 S310 mAb VL (VK)
QSALTQPASVSGSPGQSITISCTGTSSDVGSYNLVSWYQQRPGKAPELMIYEVTKRPSGLSNRFSGSKSGNTASLTISGLQAEDEADYYCCSYAGSDTVIFGGGTKVTVL

SEQ ID NO: 160 - protein, 9 aa, Artificial Sequence
  Synthetic sequence SARS-CoV-2 S310 mAb CDRL1
SSDVGSYNL

SEQ ID NO: 161 - protein, 3 aa, Artificial Sequence
  Synthetic sequence SARS-CoV-2 S310 mAb CDRL2
EVT

SEQ ID NO: 162 - protein, 10 aa, Artificial Sequence
  Synthetic sequence SARS-CoV-2 S310 mAb CDRL3
CSYAGSDTVI

SEQ ID NO: 163 - DNA, 29902 bp, betacoronavirus SARS coronavirus 2
attaaaggtttataccttcccaggtaacaaaccaaccaactttcgatctcttgtagatctgttctctaaacgaactttaaaatctgtgtggctgtcactcggctgcatgcttagtgcactcacgcagtataattaataactaattactgtcgttgacaggacacgagtaactcgtctatcttctgcaggctgcttacggtttcgtccgtgttgcagccgatcatcagcacatctaggtttcgtccgggtgtgaccgaaaggtaagatggagagccttgtccctggtttcaacgagaaaacacacgtccaactcagtttgcctgttttacaggttcgcgacgtgctcgtacgtggctttggagactccgtggaggaggtcttatcagaggccgtcaacatcttaaagatggcacttgtggcttagtagaagttgaaaaaggcgttttgcctcaacttgaacagccctatgtgttcatcaaacgttcggatgctcgaactgcacctcatggtcatgttatggttgagctggtagcagaactcgaaggcattcagtacggtcgtagtggtgagacacttggtgtccttgtccctcatgtgggcgaaataccagtggcttaccgcaaggttcttcttcgtaagaacggtaataaaggagctggtggccatagttacggcgccgatctaaagtcatttgacttaggcgacgagcttggcactgatccttatgaagattttcaagaaaactggaacactaaacatagcagtggtgttacccgtgaactcatgcgtgagcttaacggaggggcatacactcgctatgtcgataacaacttctgtggccctgatggctaccctcttgagtgcattaaagaccttctagcacgtgctggtaaagcttcatgcactttgtccgaacaactggactttattgacactaagaggggtgtatactgctgccgtgaacatgagcatgaaattgcttggtacacggaacgttctgaaaagagctatgaattgcagacaccttttgaaattaaattggcaaagaaatttgacaccttcaatggggaatgtccaaattttgtatttcccttaaattccataatcaagactattcaaccaagggttgaaaagaaaaagcttgatggctttatgggtagaattcgatctgtctatccagttgcgtcaccaaatgaatgcaaccaaatgtgcctttcaactctcatgaagtgtgatcattgtggtgaaacttcatggcagacgggcgattttgttaaagccacttgcgaattttgtggcactgagaatttgactaaagaaggtgccactacttgtggttacttaccccaaaatgctgttgttaaaatttattgtccagcatgtcacaattcagaagtaggacctgagcatagtcttgccgaataccataatgaatctggcttgaaaaccattcttcgtaagggtggtcgcactattgcctttggaggctgtgtgttctcttatgttggttgccataacaagtgtgcctattgggttccacgtgctagcgctaacataggttgtaaccatacaggtgttgttggagaaggttccgaaggtcttaatgacaaccttcttgaaatactccaaaaagagaaagtcaacatcaatattgttggtgactttaaacttaatgaagagatcgccattattttggcatctttttctgcttccacaagtgcttttgtggaaactgtgaaaggtttggattataaagcattcaaacaaattgttgaatcctgtggtaattttaaagttacaaaaggaaaagctaaaaaaggtgcctggaatattggtgaacagaaatcaatactgagtcctctttatgcatttgcatcagaggctgctcgtgttgtacgatcaattttctcccgcactcttgaaactgctcaaaattctgtgcgtgttttacagaaggccgctataacaatactagatggaatttcacagtattcactgagactcattgatgctatgatgttcacatctgatttggctactaacaatctagttgtaatggcctacattacaggtggtgttgttcagttgacttcgcagtggctaactaacatctttggcactgtttatgaaaaactcaaacccgtccttgattggcttgaagagaagtttaaggaaggtgtagagtttcttagagacggttgggaaattgttaaatttatctcaacctgtgcttgtgaaattgtcggtggacaaattgtcacctgtgcaaaggaaattaaggagagtgttcagacattctttaagcttgtaaataaatttttggctttgtgtgctgactctatcattattggtggagctaaacttaaagccttgaatttaggtgaaacatttgtcacgcactcaaagggattgtacagaaagtgtgttaaatccagagaagaaactggcctactcatgcctctaaaagccccaaaagaaattatcttcttagagggagaaacacttcccacagaagtgttaacagaggaagttgtcttgaaaactggtgatttacaaccattagaacaacctactagtgaagctgttgaagctccattggttggtacaccagtttgtattaacgggcttatgttgctcgaaatcaaagacacagaaaagtactgtgcccttgcacctaatatgatggtaacaaacaataccttcacactcaaaggcggtgcaccaacaaaggttacttttggtgatgacactgtgatagaagtgcaaggttacaagagtgtgaatatcacttttgaacttgatgaaaggattgataaagtacttaatgagaagtgctctgcctatacagttgaactcggtacagaagtaaatgagttcgcctgtgttgtggcagatgctgtcataaaaactttgcaaccagtatctgaattacttacaccactgggcattgatttagatgagtggagtatggctacatactacttatttgatgagtctggtgagtttaaattggcttcacatatgtattgttctttctaccctccagatgaggatgaagaagaaggtgattgtgaagaagaagagtttgagccatcaactcaatatgagtatggtactgaagatgattaccaaggtaaacctttggaatttggtgccacttctgctgctcttcaacctgaagaagagcaagaagaagattggttagatgatgatagtcaacaaactgttggtcaacaagacggcagtgaggacaatcagacaactactattcaaacaattgttgaggttcaacctcaattagagatggaacttacaccagttgttcagactattgaagtgaatagttttagtggttatttaaaacttactgacaatgtatacattaaaaatgcagacattgtggaagaagctaaaaaggtaaaaccaacagtggttgttaatgcagccaatgtttaccttaaacatggaggaggtgttgcaggagccttaaataaggctactaacaatgccatgcaagttgaatctgatgattacatagctactaatggaccacttaaagtgggtggtagttgtgttttaagcggacacaatcttgctaaacactgtcttcatgttgtcggcccaaatgttaacaaaggtgaagacattcaacttcttaagagtgcttatgaaaattttaatcagcacgaagttctacttgcaccattattatcagctggtatttttggtgctgaccctatacattctttaagagtttgtgtagatactgttcgcacaaatgtctacttagctgtctttgataaaaatctctatgacaaacttgtttcaagctttttggaaatgaagagtgaaaagcaagttgaacaaaagatcgctgagattcctaaagaggaagttaagccatttataactgaaagtaaaccttcagttgaacagagaaaacaagatgataagaaaatcaaagcttgtgttgaagaagttacaacaactctggaagaaactaagttcctcacagaaaacttgttactttatattgacattaatggcaatcttcatccagattctgccactcttgttagtgacattgacatcactttcttaaagaaagatgctccatatatagtgggtgatgttgttcaagagggtgttttaactgctgtggttatacctactaaaaaggctggtggcactactgaaatgctagcgaaagctttgagaaaagtgccaacagacaattatataaccacttacccgggtcagggtttaaatggttacactgtagaggaggcaaagacagtgcttaaaaagtgtaaaagtgccttttacattctaccatctattatctctaatgagaagcaagaaattcttggaactgtttcttggaatttgcgagaaatgcttgcacatgcagaagaaacacgcaaattaatgcctgtctgtgtggaaactaaagccatagtttcaactatacagcgtaaatataagggtattaaaatacaagagggtgtggttgattatggtgctagattttacttttacaccagtaaaacaactgtagcgtcacttatcaacacacttaacgatctaaatgaaactcttgttacaatgccacttggctatgtaacacatggcttaaatttggaagaagctgctcggtatatgagatctctcaaagtgccagctacagtttctgtttcttcacctgatgctgttacagcgtataatggttatcttacttcttcttctaaaacacctgaagaacattttattgaaaccatctcacttgctggttcctataaagattggtcctattctggacaatctacacaactaggtatagaatttcttaagagaggtgataaaagtgtatattacactagtaatcctaccacattccacctagatggtgaagttatcacctttgacaatcttaagacacttctttctttgagagaagtgaggactattaaggtgtttacaacagtagacaacattaacctccacacgcaagttgtggacatgtcaatgacatatggacaacagtttggtccaacttatttggatggagctgatgttactaaaataaaacctcataattcacatgaaggtaaaacattttatgttttacctaatgatgacactctacgtgttgaggcttttgagtactaccacacaactgatcctagttttctgggtaggtacatgtcagcattaaatcacactaaaaagtggaaatacccacaagttaatggtttaacttctattaaatgggcagataacaactgttatcttgccactgcattgttaacactccaacaaatagagttgaagtttaatccacctgctctacaagatgcttattacagagcaagggctggtgaagctgctaacttttgtgcacttatcttagcctactgtaataagacagtaggtgagttaggtgatgttagagaaacaatgagttacttgtttcaacatgccaatttagattcttgcaaaagagtcttgaacgtggtgtgtaaaacttgtggacaacagcagacaacccttaagggtgtagaagctgttatgtacatgggcacactttcttatgaacaatttaagaaaggtgttcagataccttgtacgtgtggtaaacaagctacaaaatatctagtacaacaggagtcaccttttgttatgatgtcagcaccacctgctcagtatgaacttaagcatggtacatttacttgtgctagtgagtacactggtaattaccagtgtggtcactataaacatataacttctaaagaaactttgtattgcatagacggtgctttacttacaaagtcctcagaatacaaaggtcctattacggatgttttctacaaagaaaacagttacacaacaaccataaaaccagttacttataaattggatggtgttgtttgtacagaaattgaccctaagttggacaattattataagaaagacaattcttatttcacagagcaaccaattgatcttgtaccaaaccaaccatatccaaacgcaagcttcgataattttaagtttgtatgtgataatatcaaatttgctgatgatttaaaccagttaactggttataagaaacctgcttcaagagagcttaaagttacatttttccctgacttaaatggtgatgtggtggctattgattataaacactacacaccctcttttaagaaaggagctaaattgttacataaacctattgtttggcatgttaacaatgcaactaataaagccacgtataaaccaaatacctggtgtatacgttgtctttggagcacaaaaccagttgaaacatcaaattcgtttgatgtactgaagtcagaggacgcgcagggaatggataatcttgcctgcgaagatctaaaaccagtctctgaagaagtagtggaaaatcctaccatacagaaagacgttcttgagtgtaatgtgaaaactaccgaagttgtaggagacattatacttaaaccagcaaataatagtttaaaaattacagaagaggttggccacacagatctaatggctgcttatgtagacaattctagtcttactattaagaaacctaatgaattatctagagtattaggtttgaaaacccttgctactcatggtttagctgctgttaatagtgtcccttgggatactatagctaattatgctaagccttttcttaacaaagttgttagtacaactactaacatagttacacggtgtttaaaccgtgtttgtactaattatatgccttatttctttactttattgctacaattgtgtacttttactagaagtacaaattctagaattaaagcatctatgccgactactatagcaaagaatactgttaagagtgtcggtaaattttgtctagaggcttcatttaattatttgaagtcacctaatttttctaaactgataaatattataatttggtttttactattaagtgtttgcctaggttctttaatctactcaaccgctgctttaggtgttttaatgtctaatttaggcatgccttcttactgtactggttacagagaaggctatttgaactctactaatgtcactattgcaacctactgtactggttctataccttgtagtgtttgtcttagtggtttagattctttagacacctatccttctttagaaactatacaaattaccatttcatcttttaaatgggatttaactgcttttggcttagttgcagagtggtttttggcatatattcttttcactaggtttttctatgtacttggattggctgcaatcatgcaattgtttttcagctattttgcagtacattttattagtaattcttggcttatgtggttaataattaatcttgtacaaatggccccgatttcagctatggttagaatgtacatcttctttgcatcattttattatgtatggaaaagttatgtgcatgttgtagacggttgtaattcatcaacttgtatgatgtgttacaaacgtaatagagcaacaagagtcgaatgtacaactattgttaatggtgttagaaggtccttttatgtctatgctaatggaggtaaaggcttttgcaaactacacaattggaattgtgttaattgtgatacattctgtgctggtagtacatttattagtgatgaagttgcgagagacttgtcactacagtttaaaagaccaataaatcctactgaccagtcttcttacatcgttgatagtgttacagtgaagaatggttccatccatctttactttgataaagctggtcaaaagacttatgaaagacattctctctctcattttgttaacttagacaacctgagagctaataacactaaaggttcattgcctattaatgttatagtttttgatggtaaatcaaaatgtgaagaatcatctgcaaaatcagcgtctgtttactacagtcagcttatgtgtcaacctatactgttactagatcaggcattagtgtctgatgttggtgatagtgcggaagttgcagttaaaatgtttgatgcttacgttaatacgttttcatcaacttttaacgtaccaatggaaaaactcaaaacactagttgcaactgcagaagctgaacttgcaaagaatgtgtccttagacaatgtcttatctacttttatttcagcagctcggcaagggtttgttgattcagatgtagaaactaaagatgttgttgaatgtcttaaattgtcacatcaatctgacatagaagttactggcgatagttgtaataactatatgctcacctataacaaagttgaaaacatgacaccccgtgaccttggtgcttgtattgactgtagtgcgcgtcatattaatgcgcaggtagcaaaaagtcacaacattgctttgatatggaacgttaaagatttcatgtcattgtctgaacaactacgaaaacaaatacgtagtgctgctaaaaagaataacttaccttttaagttgacatgtgcaactactagacaagttgttaatgttgtaacaacaaagatagcacttaagggtggtaaaattgttaataattggttgaagcagttaattaaagttacacttgtgttcctttttgttgctgctattttctatttaataacacctgttcatgtcatgtctaaacatactgacttttcaagtgaaatcataggatacaaggctattgatggtggtgtcactcgtgacatagcatctacagatacttgttttgctaacaaacatgctgattttgacacatggtttagccagcgtggtggtagttatactaatgacaaagcttgcccattgattgctgcagtcataacaagagaagtgggttttgtcgtgcctggtttgcctggcacgatattacgcacaactaatggtgactttttgcatttcttacctagagtttttagtgcagttggtaacatctgttacacaccatcaaaacttatagagtacactgactttgcaacatcagcttgtgttttggctgctgaatgtacaatttttaaagatgcttctggtaagccagtaccatattgttatgataccaatgtactagaaggttctgttgcttatgaaagtttacgccctgacacacgttatgtgctcatggatggctctattattcaatttcctaacacctaccttgaaggttctgttagagtggtaacaacttttgattctgagtactgtaggcacggcacttgtgaaagatcagaagctggtgtttgtgtatctactagtggtagatgggtacttaacaatgattattacagatctttaccaggagttttctgtggtgtagatgctgtaaatttacttactaatatgtttacaccactaattcaacctattggtgctttggacatatcagcatctatagtagctggtggtattgtagctatcgtagtaacatgccttgcctactattttatgaggtttagaagagcttttggtgaatacagtcatgtagttgcctttaatactttactattccttatgtcattcactgtactctgtttaacaccagtttactcattcttacctggtgtttattctgttatttacttgtacttgacattttatcttactaatgatgtttcttttttagcacatattcagtggatggttatgttcacacctttagtacctttctggataacaattgcttatatcatttgtatttccacaaagcatttctattggttctttagtaattacctaaagagacgtgtagtctttaatggtgtttcctttagtacttttgaagaagctgcgctgtgcacctttttgttaaataaagaaatgtatctaaagttgcgtagtgatgtgctattacctcttacgcaatataatagatacttagctctttataataagtacaagtattttagtggagcaatggatacaactagctacagagaagctgcttgttgtcatctcgcaaaggctctcaatgacttcagtaactcaggttctgatgttctttaccaaccaccacaaacctctatcacctcagctgttttgcagagtggttttagaaaaatggcattcccatctggtaaagttgagggttgtatggtacaagtaacttgtggtacaactacacttaacggtctttggcttgatgacgtagtttactgtccaagacatgtgatctgcacctctgaagacatgcttaaccctaattatgaagatttactcattcgtaagtctaatcataatttcttggtacaggctggtaatgttcaactcagggttattggacattctatgcaaaattgtgtacttaagcttaaggttgatacagccaatcctaagacacctaagtataagtttgttcgcattcaaccaggacagactttttcagtgttagcttgttacaatggttcaccatctggtgtttaccaatgtgctatgaggcccaatttcactattaagggttcattccttaatggttcatgtggtagtgttggttttaacatagattatgactgtgtctctttttgttacatgcaccatatggaattaccaactggagttcatgctggcacagacttagaaggtaacttttatggaccttttgttgacaggcaaacagcacaagcagctggtacggacacaactattacagttaatgttttagcttggttgtacgctgctgttataaatggagacaggtggtttctcaatcgatttaccacaactcttaatgactttaaccttgtggctatgaagtacaattatgaacctctaacacaagaccatgttgacatactaggacctctttctgctcaaactggaattgccgttttagatatgtgtgcttcattaaaagaattactgcaaaatggtatgaatggacgtaccatattgggtagtgctttattagaagatgaatttacaccttttgatgttgttagacaatgctcaggtgttactttccaaagtgcagtgaaaagaacaatcaagggtacacaccactggttgttactcacaattttgacttcacttttagttttagtccagagtactcaatggtctttgttcttttttttgtatgaaaatgcctttttaccttttgctatgggtattattgctatgtctgcttttgcaatgatgtttgtcaaacataagcatgcatttctctgtttgtttttgttaccttctcttgccactgtagcttattttaatatggtctatatgcctgctagttgggtgatgcgtattatgacatggttggatatggttgatactagtttgtctggttttaagctaaaagactgtgttatgtatgcatcagctgtagtgttactaatccttatgacagcaagaactgtgtatgatgatggtgctaggagagtgtggacacttatgaatgtcttgacactcgtttataaagtttattatggtaatgctttagatcaagccatttccatgtgggctcttataatctctgttacttctaactactcaggtgtagttacaactgtcatgtttttggccagaggtattgtttttatgtgtgttgagtattgccctattttcttcataactggtaatacacttcagtgtataatgctagtttattgtttcttaggctatttttgtacttgttactttggcctcttttgtttactcaaccgctactttagactgactcttggtgtttatgattacttagtttctacacaggagtttagatatatgaattcacagggactactcccacccaagaatagcatagatgccttcaaactcaacattaaattgttgggtgttggtggcaaaccttgtatcaaagtagccactgtacagtctaaaatgtcagatgtaaagtgcacatcagtagtcttactctcagttttgcaacaactcagagtagaatcatcatctaaattgtgggctcaatgtgtccagttacacaatgacattctcttagctaaagatactactgaagcctttgaaaaaatggtttcactactttctgttttgctttccatgcagggtgctgtagacataaacaagctttgtgaagaaatgctggacaacagggcaaccttacaagctatagcctcagagtttagttcccttccatcatatgcagcttttgctactgctcaagaagcttatgagcaggctgttgctaatggtgattctgaagttgttcttaaaaagttgaagaagtctttgaatgtggctaaatctgaatttgaccgtgatgcagccatgcaacgtaagttggaaaagatggctgatcaagctatgacccaaatgtataaacaggctagatctgaggacaagagggcaaaagttactagtgctatgcagacaatgcttttcactatgcttagaaagttggataatgatgcactcaacaacattatcaacaatgcaagagatggttgtgttcccttgaacataatacctcttacaacagcagccaaactaatggttgtcataccagactataacacatataaaaatacgtgtgatggtacaacatttacttatgcatcagcattgtgggaaatccaacaggttgtagatgcagatagtaaaattgttcaacttagtgaaattagtatggacaattcacctaatttagcatggcctcttattgtaacagctttaagggccaattctgctgtcaaattacagaataatgagcttagtcctgttgcactacgacagatgtcttgtgctgccggtactacacaaactgcttgcactgatgacaatgcgttagcttactacaacacaacaaagggaggtaggtttgtacttgcactgttatccgatttacaggatttgaaatgggctagattccctaagagtgatggaactggtactatctatacagaactggaaccaccttgtaggtttgttacagacacacctaaaggtcctaaagtgaagtatttatactttattaaaggattaaacaacctaaatagaggtatggtacttggtagtttagctgccacagtacgtctacaagctggtaatgcaacagaagtgcctgccaattcaactgtattatctttctgtgcttttgctgtagatgctgctaaagcttacaaagattatctagctagtgggggacaaccaatcactaattgtgttaagatgttgtgtacacacactggtactggtcaggcaataacagttacaccggaagccaatatggatcaagaatcctttggtggtgcatcgtgttgtctgtactgccgttgccacatagatcatccaaatcctaaaggattttgtgacttaaaaggtaagtatgtacaaatacctacaacttgtgctaatgaccctgtgggttttacacttaaaaacacagtctgtaccgtctgcggtatgtggaaaggttatggctgtagttgtgatcaactccgcgaacccatgcttcagtcagctgatgcacaatcgtttttaaacgggtttgcggtgtaagtgcagcccgtcttacaccgtgcggcacaggcactagtactgatgtcgtatacagggcttttgacatctacaatgataaagtagctggttttgctaaattcctaaaaactaattgttgtcgcttccaagaaaaggacgaagatgacaatttaattgattcttactttgtagttaagagacacactttctctaactaccaacatgaagaaacaatttataatttacttaaggattgtccagctgttgctaaacatgacttctttaagtttagaatagacggtgacatggtaccacatatatcacgtcaacgtcttactaaatacacaatggcagacctcgtctatgctttaaggcattttgatgaaggtaattgtgacacattaaaagaaatacttgtcacatacaattgttgtgatgatgattatttcaataaaaaggactggtatgattttgtagaaaacccagatatattacgcgtatacgccaacttaggtgaacgtgtacgccaagctttgttaaaaacagtacaattctgtgatgccatgcgaaatgctggtattgttggtgtactgacattagataatcaagatctcaatggtaactggtatgatttcggtgatttcatacaaaccacgccaggtagtggagttcctgttgtagattcttattattcattgttaatgcctatattaaccttgaccagggctttaactgcagagtcacatgttgacactgacttaacaaagccttacattaagtgggatttgttaaaatatgacttcacggaagagaggttaaaactctttgaccgttattttaaatattgggatcagacataccacccaaattgtgttaactgtttggatgacagatgcattctgcattgtgcaaactttaatgttttattctctacagtgttcccacctacaagttttggaccactagtgagaaaaatatttgttgatggtgttccatttgtagtttcaactggataccacttcagagagctaggtgttgtacataatcaggatgtaaacttacatagctctagacttagttttaaggaattacttgtgtatgctgctgaccctgctatgcacgctgcttctggtaatctattactagataaacgcactacgtgcttttcagtagctgcacttactaacaatgttgcttttcaaactgtcaaacccggtaattttaacaaagacttctatgactttgctgtgtctaagggtttctttaaggaaggaagttctgttgaattaaaacacttcttctttgctcaggatggtaatgctgctatcagcgattatgactactatcgttataatctaccaacaatgtgtgatatcagacaactactatttgtagttgaagttgttgataagtactttgattgttacgatggtggctgtattaatgctaaccaagtcatcgtcaacaacctagacaaatcagctggttttccatttaataaatggggtaaggctagactttattatgattcaatgagttatgaggatcaagatgcacttttcgcatatacaaaacgtaatgtcatccctactataactcaaatgaatcttaagtatgccattagtgcaaagaatagagctcgcaccgtagctggtgtctctatctgtagtactatgaccaatagacagtttcatcaaaaattattgaaatcaatagccgccactagaggagctactgtagtaattggaacaagcaaattctatggtggttggcacaacatgttaaaaactgtttatagtgatgtagaaaaccctcaccttatgggttgggattatcctaaatgtgatagagccatgcctaacatgcttagaattatggcctcacttgttcttgctcgcaaacatacaacgtgttgtagcttgtcacaccgtttctatagattagctaatgagtgtgctcaagtattgagtgaaatggtcatgtgtggcggttcactatatgttaaaccaggtggaacctcatcaggagatgccacaactgcttatgctaatagtgtttttaacatttgtcaagctgtcacggccaatgttaatgcacttttatctactgatggtaacaaaattgccgataagtatgtccgcaatttacaacacagactttatgagtgtctctatagaaatagagatgttgacacagactttgtgaatgagttttacgcatatttgcgtaaacatttctcaatgatgatactctctgacgatgctgttgtgtgtttcaatagcacttatgcatctcaaggtctagtggctagcataaagaactttaagtcagttctttattatcaaaacaatgtttttatgtctgaagcaaaatgttggactgagactgaccttactaaaggacctcatgaattttgctctcaacatacaatgctagttaaacagggtgatgattatgtgtaccttccttacccagatccatcaagaatcctaggggccggctgttttgtagatgatatcgtaaaaacagatggtacacttatgattgaacggttcgtgtctttagctatagatgcttacccacttactaaacatcctaatcaggagtatgctgatgtctttcatttgtacttacaatacataagaaagctacatgatgagttaacaggacacatgttagacatgtattctgttatgcttactaatgataacacttcaaggtattgggaacctgagttttatgaggctatgtacacaccgcatacagtcttacaggctgttggggcttgtgttctttgcaattcacagacttcattaagatgtggtgcttgcatacgtagaccattcttatgttgtaaatgctgttacgaccatgtcatatcaacatcacataaattagtcttgtctgttaatccgtatgtttgcaatgctccaggttgtgatgtcacagatgtgactcaactttacttaggaggtatgagctattattgtaaatcacataaaccacccattagttttccattgtgtgctaatggacaagtttttggtttatataaaaatacatgtgttggtagcgataatgttactgactttaatgcaattgcaacatgtgactggacaaatgctggtgattacattttagctaacacctgtactgaaagactcaagctttttgcagcagaaacgctcaaagctactgaggagacatttaaactgtcttatggtattgctactgtacgtgaagtgctgtctgacagagaattacatctttcatgggaagttggtaaacctagaccaccacttaaccgaaattatgtctttactggttatcgtgtaactaaaaacagtaaagtacaaataggagagtacacctttgaaaaaggtgactatggtgatgctgttgtttaccgaggtacaacaacttacaaattaaatgttggtgattattttgtgctgacatcacatacagtaatgccattaagtgcacctacactagtgccacaagagcactatgttagaattactggcttatacccaacactcaatatctcagatgagttttctagcaatgttgcaaattatcaaaaggttggtatgcaaaagtattctacactccagggaccacctggtactggtaagagtcattttgctattggcctagctctctactacccttctgctcgcatagtgtatacagcttgctctcatgccgctgttgatgcactatgtgagaaggcattaaaatatttgcctatagataaatgtagtagaattatacctgcacgtgctcgtgtagagtgttttgataaattcaaagtgaattcaacattagaacagtatgtcttttgtactgtaaatgcattgcctgagacgacagcagatatagttgtctttgatgaaatttcaatggccacaaattatgatttgagtgttgtcaatgccagattacgtgctaagcactatgtgtacattggcgaccctgctcaattacctgcaccacgcacattgctaactaagggcacactagaaccagaatatttcaattcagtgtgtagacttatgaaaactataggtccagacatgttcctcggaacttgtcggcgttgtcctgctgaaattgttgacactgtgagtgctttggtttatgataataagcttaaagcacataaagacaaatcagctcaatgctttaaaatgttttataagggtgttatcacgcatgatgtttcatctgcaattaacaggccacaaataggcgtggtaagagaattccttacacgtaaccctgcttggagaaaagctgtctttatttcaccttataattcacagaatgctgtagcctcaaagattttgggactaccaactcaaactgttgattcatcacagggctcagaatatgactatgtcatattcactcaaaccactgaaacagctcactcttgtaatgtaaacagatttaatgttgctattaccagagcaaaagtaggcatactttgcataatgtctgatagagacctttatgacaagttgcaatttacaagtcttgaaattccacgtaggaatgtggcaactttacaagctgaaaatgtaacaggactctttaaagattgtagtaaggtaatcactgggttacatcctacacaggcacctacacacctcagtgttgacactaaattcaaaactgaaggtttatgtgttgacatacctggcatacctaaggacatgacctatagaagactcatctctatgatgggttttaaaatgaattatcaagttaatggttaccctaacatgtttatcacccgcgaagaagctataagacatgtacgtgcatggattggcttcgatgtcgaggggtgtcatgctactagagaagctgttggtaccaatttacctttacagctaggtttttctacaggtgttaacctagttgctgtacctacaggttatgttgatacacctaataatacagatttttccagagttagtgctaaaccaccgcctggagatcaatttaaacacctcataccacttatgtacaaaggacttccttggaatgtagtgcgtataaagattgtacaaatgttaagtgacacacttaaaaatctctctgacagagtcgtatttgtcttatgggcacatggctttgagttgacatctatgaagtattttgtgaaaataggacctgagcgcacctgttgtctatgtgatagacgtgccacatgcttttccactgcttcagacacttatgcctgttggcatcattctattggatttgattacgtctataatccgtttatgattgatgttcaacaatggggttttacaggtaacctacaaagcaaccatgatctgtattgtcaagtccatggtaatgcacatgtagctagttgtgatgcaatcatgactaggtgtctagctgtccacgagtgctttgttaagcgtgttgactggactattgaatatcctataattggtgatgaactgaagattaatgcggcttgtagaaaggttcaacacatggttgttaaagctgcattattagcagacaaattcccagttcttcacgacattggtaaccctaaagctattaagtgtgtacctcaagctgatgtagaatggaagttctatgatgcacagccttgtagtgacaaagcttataaaatagaagaattattctattcttatgccacacattctgacaaattcacagatggtgtatgcctattttggaattgcaatgtcgatagatatcctgctaattccattgtttgtagatttgacactagagtgctatctaaccttaacttgcctggttgtgatggtggcagtttgtatgtaaataaacatgcattccacacaccagcttttgataaaagtgcttttgttaatttaaaacaattaccatttttctattactctgacagtccatgtgagtctcatggaaaacaagtagtgtcagatatagattatgtaccactaaagtctgctacgtgtataacacgttgcaatttaggtggtgctgtctgtagacatcatgctaatgagtacagattgtatctcgatgcttataacatgatgatctcagctggctttagcttgtgggtttacaaacaatttgatacttataacctctggaacacttttacaagacttcagagtttagaaaatgtggcttttaatgttgtaaataagggacactttgatggacaacagggtgaagtaccagtttctatcattaataacactgtttacacaaaagttgatggtgttgatgtagaattgtttgaaaataaaacaacattacctgttaatgtagcatttgagctttgggctaagcgcaacattaaaccagtaccagaggtgaaaatactcaataatttgggtgtggacattgctgctaatactgtgatctgggactacaaaagagatgctccagcacatatatctactattggtgtttgttctatgactgacatagccaagaaaccaactgaaacgatttgtgcaccactcactgtcttttttgatggtagagttgatggtcaagtagacttatttagaaatgcccgtaatggtgttcttattacagaaggtagtgttaaaggtttacaaccatctgtaggtcccaaacaagctagtcttaatggagtcacattaattggagaagccgtaaaaacacagttcaattattataagaaagttgatggtgttgtccaacaattacctgaaacttactttactcagagtagaaatttacaagaatttaaacccaggagtcaaatggaaattgatttcttagaattagctatggatgaattcattgaacggtataaattagaaggctatgccttcgaacatatcgtttatggagattttagtcatagtcagttaggtggtttacatctactgattggactagctaaacgttttaaggaatcaccttttgaattagaagattttattcctatggacagtacagttaaaaactatttcataacagatgcgcaaacaggttcatctaagtgtgtgtgttctgttattgatttattacttgatgattttgttgaaataataaaatcccaagatttatctgtagtttctaaggttgtcaaagtgactattgactatacagaaatttcatttatgctttggtgtaaagatggccatgtagaaacattttacccaaaattacaatctagtcaagcgtggcaaccgggtgttgctatgcctaatctttacaaaatgcaaagaatgctattagaaaagtgtgaccttcaaaattatggtgatagtgcaacattacctaaaggcataatgatgaatgtcgcaaaatatactcaactgtgtcaatatttaaacacattaacattagctgtaccctataatatgagagttatacattttggtgctggttctgataaaggagttgcaccaggtacagctgttttaagacagtggttgcctacgggtacgctgcttgtcgattcagatcttaatgactttgtctctgatgcagattcaactttgattggtgattgtgcaactgtacatacagctaataaatgggatctcattattagtgatatgtacgaccctaagactaaaaatgttacaaaagaaaatgactctaaagagggttttttcacttacatttgtgggtttatacaacaaaagctagctcttggaggttccgtggctataaagataacagaacattcttggaatgctgatctttataagctcatgggacacttcgcatggtggacagcctttgttactaatgtgaatgcgtcatcatctgaagcatttttaattggatgtaattatcttggcaaaccacgcgaacaaatagatggttatgtcatgcatgcaaattacatattttggaggaatacaaatccaattcagttgtcttcctattctttatttgacatgagtaaatttccccttaaattaaggggtactgctgttatgtctttaaaagaaggtcaaatcaatgatatgattttatctcttcttagtaaaggtagacttataattagagaaaacaacagagttgttatttctagtgatgttcttgttaacaactaaacgaacaatgtttgtttttcttgttttattgccactagtctctagtcagtgtgttaatcttacaaccagaactcaattaccccctgcatacactaattctttcacacgtggtgtttattaccctgacaaagttttcagatcctcagttttacattcaactcaggacttgttcttacctttcttttccaatgttacttggttccatgctatacatgtctctgggaccaatggtactaagaggtttgataaccctgtcctaccatttaatgatggtgtttattttgcttccactgagaagtctaacataataagaggctggatttttggtactactttagattcgaagacccagtccctacttattgttaataacgctactaatgttgttattaaagtctgtgaatttcaattttgtaatgatccatttttgggtgtttattaccacaaaaacaacaaaagttggatggaaagtgagttcagagtttattctagtgcgaataattgcacttttgaatatgtctctcagccttttcttatggaccttgaaggaaaacagggtaatttcaaaaatcttagggaatttgtgtttaagaatattgatggttattttaaaatatattctaagcacacgcctattaatttagtgcgtgatctccctcagggtttttcggctttagaaccattggtagatttgccaataggtattaacatcactaggtttcaaactttacttgctttacatagaagttatttgactcctggtgattcttcttcaggttggacagctggtgctgcagcttattatgtgggttatcttcaacctaggacttttctattaaaatataatgaaaatggaaccattacagatgctgtagactgtgcacttgaccctctctcagaaacaaagtgtacgttgaaatccttcactgtagaaaaaggaatctatcaaacttctaactttagagtccaaccaacagaatctattgttagatttcctaatattacaaacttgtgcccttttggtgaagtttttaacgccaccagatttgcatctgtttatgcttggaacaggaagagaatcagcaactgtgttgctgattattctgtcctatataattccgcatcattttccacttttaagtgttatggagtgtctcctactaaattaaatgatctctgctttactaatgtctatgcagattcatttgtaattagaggtgatgaagtcagacaaatcgctccagggcaaactggaaagattgctgattataattataaattaccagatgattttacaggctgcgttatagcttggaattctaacaatcttgattctaaggttggtggtaattataattacctgtatagattgtttaggaagtctaatctcaaaccttttgagagagatatttcaactgaaatctatcaggccggtagcacaccttgtaatggtgttgaaggttttaattgttactttcctttacaatcatatggtttccaacccactaatggtgttggttaccaaccatacagagtagtagtactttcttttgaacttctacatgcaccagcaactgtttgtggacctaaaaagtctactaatttggttaaaaacaaatgtgtcaatttcaacttcaatggtttaacaggcacaggtgttcttactgagtctaacaaaaagtttctgcctttccaacaatttggcagagacattgctgacactactgatgctgtccgtgatccacagacacttgagattcttgacattacaccatgttcttttggtggtgtcagtgttataacaccaggaacaaatacttctaaccaggttgctgttctttatcaggatgttaactgcacagaagtccctgttgctattcatgcagatcaacttactcctacttggcgtgtttattctacaggttctaatgtttttcaaacacgtgcaggctgtttaataggggctgaacatgtcaacaactcatatgagtgtgacatacccattggtgcaggtatatgcgctagttatcagactcagactaattctcctcggcgggcacgtagtgtagctagtcaatccatcattgcctacactatgtcacttggtgcagaaaattcagttgcttactctaataactctattgccatacccacaaattttactattagtgttaccacagaaattctaccagtgtctatgaccaagacatcagtagattgtacaatgtacatttgtggtgattcaactgaatgcagcaatcttttgttgcaatatggcagtttttgtacacaattaaaccgtgctttaactggaatagctgttgaacaagacaaaaacacccaagaagtttttgcacaagtcaaacaaatttacaaaacaccaccaattaaagattttggtggttttaatttttcacaaatattaccagatccatcaaaaccaagcaagaggtcatttattgaagatctacttttcaacaaagtgacacttgcagatgctggcttcatcaaacaatatggtgattgccttggtgatattgctgctagagacctcatttgtgcacaaaagtttaacggccttactgttttgccacctttgctcacagatgaaatgattgctcaatacacttctgcactgttagcgggtacaatcacttctggttggacctttggtgcaggtgctgcattacaaataccatttgctatgcaaatggcttataggtttaatggtattggagttacacagaatgttctctatgagaaccaaaaattgattgccaaccaatttaatagtgctattggcaaaattcaagactcactttcttccacagcaagtgcacttggaaaacttcaagatgtggtcaaccaaaatgcacaagctttaaacacgcttgttaaacaacttagctccaattttggtgcaatttcaagtgttttaaatgatatcctttcacgtcttgacaaagttgaggctgaagtgcaaattgataggttgatcacaggcagacttcaaagtttgcagacatatgtgactcaacaattaattagagctgcagaaatcagagcttctgctaatcttgctgctactaaaatgtcagagtgtgtacttggacaatcaaaaagagttgatttttgtggaaagggctatcatcttatgtccttccctcagtcagcacctcatggtgtagtcttcttgcatgtgacttatgtccctgcacaagaaaagaacttcacaactgctcctgccatttgtcatgatggaaaagcacactttcctcgtgaaggtgtctttgtttcaaatggcacacactggtttgtaacacaaaggaatttttatgaaccacaaatcattactacagacaacacatttgtgtctggtaactgtgatgttgtaataggaattgtcaacaacacagtttatgatcctttgcaacctgaattagactcattcaaggaggagttagataaatattttaagaatcatacatcaccagatgttgatttaggtgacatctctggcattaatgcttcagttgtaaacattcaaaaagaaattgaccgcctcaatgaggttgccaagaatttaaatgaatctctcatcgatctccaagaacttggaaagtatgagcagtatataaaatggccatggtacatttggctaggttttatagctggcttgattgccatagtaatggtgacaattatgctttgctgtatgaccagttgctgtagttgtctcaagggctgttgttcttgtggatcctgctgcaaatttgatgaagacgactctgagccagtgctcaaaggagtcaaattacattacacataaacgaacttatggatttgtttatgagaatcttcacaattggaactgtaactttgaagcaaggtgaaatcaaggatgctactccttcagattttgttcgcgctactgcaacgataccgatacaagcctcactccctttcggatggcttattgttggcgttgcacttcttgctgtttttcagagcgcttccaaaatcataaccctcaaaaagagatggcaactagcactctccaagggtgttcactttgtttgcaacttgctgttgttgtttgtaacagtttactcacaccttttgctcgttgctgctggccttgaagccccttttctctatctttatgctttagtctacttcttgcagagtataaactttgtaagaataataatgaggctttggctttgctggaaatgccgttccaaaaacccattactttatgatgccaactattttctttgctggcatactaattgttacgactattgtataccttacaatagtgtaacttcttcaattgtcattacttcaggtgatggcacaacaagtcctatttctgaacatgactaccagattggtggttatactgaaaaatgggaatctggagtaaaagactgtgttgtattacacagttacttcacttcagactattaccagctgtactcaactcaattgagtacagacactggtgttgaacatgttaccttcttcatctacaataaaattgttgatgagcctgaagaacatgtccaaattcacacaatcgacggttcatccggagttgttaatccagtaatggaaccaatttatgatgaaccgacgacgactactagcgtgcctttgtaagcacaagctgatgagtacgaacttatgtactcattcgtttcggaagagacaggtacgttaatagttaatagcgtacttctttttcttgctttcgtggtattcttgctagttacactagccatccttactgcgcttcgattgtgtgcgtactgctgcaatattgttaacgtgagtcttgtaaaaccttctttttacgtttactctcgtgttaaaaatctgaattcttctagagttcctgatcttctggtctaaacgaactaaatattatattagtttttctgtttggaactttaattttagccatggcagattccaacggtactattaccgttgaagagcttaaaaagctccttgaacaatggaacctagtaataggtttcctattccttacatggatttgtcttctacaatttgcctatgccaacaggaataggtttttgtatataattaagttaattttcctctggctgttatggccagtaactttagcttgttttgtgcttgctgctgtttacagaataaattggatcaccggtggaattgctatcgcaatggcttgtcttgtaggcttgatgtggctcagctacttcattgcttctttcagactgtttgcgcgtacgcgttccatgtggtcattcaatccagaaactaacattcttctcaacgtgccactccatggcactattctgaccagaccgcttctagaaagtgaactcgtaatcggagctgtgatccttcgtggacatcttcgtattgctggacaccatctaggacgctgtgacatcaaggacctgcctaaagaaatcactgttgctacatcacgaacgctttcttattacaaattgggagcttcgcagcgtgtagcaggtgactcaggttttgctgcatacagtcgctacaggattggcaactataaattaaacacagaccattccagtagcagtgacaatattgctttgcttgtacagtaagtgacaacagatgtttcatctcgttgactttcaggttactatagcagagatattactaattattatgaggacttttaaagtttccatttggaatcttgattacatcataaacctcataattaaaaatttatctaagtcactaactgagaataaatattctcaattagatgaagagcaaccaatggagattgattaaacgaacatgaaaattattcttttcttggcactgataacactcgctacttgtgagctttatcactaccaagagtgtgttagaggtacaacagtacttttaaaagaaccttgctcttctggaacatacgagggcaattcaccatttcatcctctagctgataacaaatttgcactgacttgctttagcactcaatttgcttttgcttgtcctgacggcgtaaaacacgtctatcagttacgtgccagatcagtttcacctaaactgttcatcagacaagaggaagttcaagaactttactctccaatttttcttattgttgcggcaatagtgtttataacactttgcttcacactcaaaagaaagacagaatgattgaactttcattaattgacttctatttgtgctttttagcctttctgctattccttgttttaattatgcttattatcttttggttctcacttgaactgcaagatcataatgaaacttgtcacgcctaaacgaacatgaaatttcttgttttcttaggaatcatcacaactgtagctgcatttcaccaagaatgtagtttacagtcatgtactcaacatcaaccatatgtagttgatgacccgtgtcctattcacttctattctaaatggtatattagagtaggagctagaaaatcagcacctttaattgaattgtgcgtggatgaggctggttctaaatcacccattcagtacatcgatatcggtaattatacagtttcctgtttaccttttacaattaattgccaggaacctaaattgggtagtcttgtagtgcgttgttcgttctatgaagactttttagagtatcatgacgttcgtgttgttttagatttcatctaaacgaacaaactaaaatgtctgataatggaccccaaaatcagcgaaatgcaccccgcattacgtttggtggaccctcagattcaactggcagtaaccagaatggagaacgcagtggggcgcgatcaaaacaacgtcggccccaaggtttacccaataatactgcgtcttggttcaccgctctcactcaacatggcaaggaagaccttaaattccctcgaggacaaggcgttccaattaacaccaatagcagtccagatgaccaaattggctactaccgaagagctaccagacgaattcgtggtggtgacggtaaaatgaaagatctcagtccaagatggtatttctactacctaggaactgggccagaagctggacttccctatggtgctaacaaagacggcatcatatgggttgcaactgagggagccttgaatacaccaaaagatcacattggcacccgcaatcctgctaacaatgctgcaatcgtgctacaacttcctcaaggaacaacattgccaaaaggcttctacgcagaagggagcagaggcggcagtcaagcctcttctcgttcctcatcacgtagtcgcaacagttcaagaaattcaactccaggcagcagtaggggaacttctcctgctagaatggctggcaatggcggtgatgctgctcttgctttgctgctgcttgacagattgaaccagcttgagagcaaaatgtctggtaaaggccaacaacaacaaggccaaactgtcactaagaaatctgctgctgaggcttctaagaagcctcggcaaaaacgtactgccactaaagcatacaatgtaacacaagctttcggcagacgtggtccagaacaaacccaaggaaattttggggaccaggaactaatcagacaaggaactgattacaaacattggccgcaaattgcacaatttgcccccagcgcttcagcgttcttcggaatgtcgcgcattggcatggaagtcacaccttcgggaacgtggttgacctacacaggtgccatcaaattggatgacaaagatccaaatttcaaagatcaagtcattttgctgaataagcatattgacgcatacaaaacattcccaccaacagagcctaaaaaggacaaaaagaagaaggctgatgaaactcaagccttaccgcagagacagaagaaacagcaaactgtgactcttcttcctgctgcagatttggatgatttctccaaacaattgcaacaatccatgagcagtgctgactcaactcaggcctaaactcatgcagaccacacaaggcagatgggctatataaacgttttcgcttttccgtttacgatatatagtctactcttgtgcagaatgaattctcgtaactacatagcacaagtagatgtagttaactttaatctcacatagcaatctttaatcagtgtgtaacattagggaggacttgaaagagccaccacattttcaccgaggccacgcggagtacgatcgagtgtacagtgaacaatgctagggagagctgcctatatggaagagccctaatgtgtaaaattaattttagtagtgctatccccatgtgattttaatagcttcttaggagaatgacaaaaaaaaaaaaaaaaaaaaaaaaaaaaaaaaa

SEQ ID NO: 164 - protein, 7096 aa, betacoronavirus SARS coronavirus 2 [sequence omitted]

SEQ ID NO: 165 - protein, 1273 aa, betacoronavirus SARS coronavirus 2
MFVFLVLLPLVSSQCVNLTTRTQLPPAYTNSFTRGVYYPDKVFRSSVLHSTQDLFLPFFSNVTWFHAIHVSGTNGTKRFDNPVLPFNDGVYFASTEKSNIIRGWIFGTTLDSKTQSLLIVNNATNVVIKVCEFQFCNDPFLGVYYHKNNKSWMESEFRVYSSANNCTFEYVSQPFLMDLEGKQGNFKNLREFVFKNIDGYFKIYSKHTPINLVRDLPQGFSALEPLVDLPIGINITRFQTLLALHRSYLTPGDSSSGWTAGAAAYYVGYLQPRTFLLKYNENGTITDAVDCALDPLSETKCTLKSFTVEKGIYQTSNFRVQPTESIVRFPNITNLCPFGEVFNATRFASVYAWNRKRISNCVADYSVLYNSASFSTFKCYGVSPTKLNDLCFTNVYADSFVIRGDEVRQIAPGQTGKIADYNYKLPDDFTGCVIAWNSNNLDSKVGGNYNYLYRLFRKSNLKPFERDISTEIYQAGSTPCNGVEGFNCYFPLQSYGFQPTNGVGYQPYRVVVLSFELLHAPATVCGPKKSTNLVKNKCVNFNFNGLTGTGVLTESNKKFLPFQQFGRDIADTTDAVRDPQTLEILDITPCSFGGVSVITPGTNTSNQVAVLYQDVNCTEVPVAIHADQLTPTWRVYSTGSNVFQTRAGCLIGAEHVNNSYECDIPIGAGICASYQTQTNSPRRARSVASQSIIAYTMSLGAENSVAYSNNSIAIPTNFTISVTTEILPVSMTKTSVDCTMYICGDSTECSNLLLQYGSFCTQLNRALTGIAVEQDKNTQEVFAQVKQIYKTPPIKDFGGFNFSQILPDPSKPSKRSFIEDLLFNKVTLADAGFIKQYGDCLGDIAARDLICAQKFNGLTVLPPLLTDEMIAQYTSALLAGTITSGWTFGAGAALQIPFAMQMAYRFNGIGVTQNVLYENQKLIANQFNSAIGKIQDSLSSTASALGKLQDVVNQNAQALNTLVKQLSSNFGAISSVLNDILSRLDKVEAEVQIDRLITGRLQSLQTYVTQQLIRAAEIRASANLAATKMSECVLGQSKRVDFCGKGYHLMSFPQSAPHGVVFLHVTYVPAQEKNFTTAPAICHDGKAHFPREGVFVSNGTHWFVTQRNFYEPQIITTDNTFVSGNCDVVIGIVNNTVYDPLQPELDSFKEELDKYFKNHTSPDVDLGDISGINASVVNIQKEIDRLNEVAKNLNESLIDLQELGKYEQYIKWPWYIWLGFIAGLIAIVMVTIMLCCMTSCCSCLKGCCSCGSCCKFDEDDSEPVLKGVKLHYT

SEQ ID NO: 166 - protein, 220 aa, Artificial Sequence
  surface glycoprotein RBD [Wuhan seafood market pneumonia virus]
NITNLCPFGEVFNATRFASVYAWNRKRISNCVADYSVLYNSASFSTFKCYGVSPTKLNDLCFTNVYADSFVIRGDEVRQIAPGQTGKIADYNYKLPDDFTGCVIAWNSNNLDSKVGGNYNYLYRLFRKSNLKPFERDISTEIYQAGSTPCNGVEGFNCYFPLQSYGFQPTNGVGYQPYRVVVLSFELLHAPATVCGPKKSTNLVKNKCVNFNFNGLTGTG

SEQ ID NO: 167 - protein, 72 aa, Artificial Sequence
  Receptor Binding Motif (RBM) in surface glycoprotein RBD [Wuhan seafood market pneumonia virus]
NSNNLDSKVGGNYNYLYRLFRKSNLKPFERDISTEIYQAGSTPCNGVEGFNCYFPLQSYGFQPTNGVGYQPY

SEQ ID NO: 168 - protein, 107 aa, Artificial Sequence [sequence omitted]

SEQ ID NO: 169 - protein, 7 aa, Artificial Sequence
  SARS-CoV-2 S309-v13 mAb CDRL1
QTVSSTS

SEQ ID NO: 170 - protein, 3 aa, Artificial Sequence
  SARS-CoV-2 S309-v13 mAb CDRL2
GAS

SEQ ID NO: 171 - protein, 8 aa, Artificial Sequence
  SARS-CoV-2 S309-v13 mAb CDRL3
QQHDTSLT

SEQ ID NO: 172 - protein, 127 aa, Artificial Sequence
  SARS-CoV-2 S309-v2.9 mAb VH
QVQLVQSGAEVKKPGASVKVSCKASGYPFTSYGISWVRQAPGQGLEWMGFISTYNANTNYAQKFQGRVTMTTDTSTTTGYMELRRLRSDDTAVYYCARDYTRGAFFGESLIGGFDNWGQGTLVTVSS

SEQ ID NO: 173 - protein, 330 aa, Artificial Sequence
  SARS-CoV-2 CH1-CH3 G1m17; IgG1*01 LS
ASTKGPSVFPLAPSSKSTSGGTAALGCLVKDYFPEPVTVSWNSGALTSGVHTFPAVLQSSGLYSLSSVVTVPSSSLGTQTYICNVNHKPSNTKVDKKVEPKSCDKTHTCPPCPAPELLGGPSVFLFPPKPKDTLMISRTPEVTCVVVDVSHEDPEVKFNWYVDGVEVHNAKTKPREEQYNSTYRVVSVLTVLHQDWLNGKEYKCKVSNKALPAPIEKTISKAKGQPREPQVYTLPPSRDELTKNQVSLTCLVKGFYPSDIAVEWESNGQPENNYKTTPPVLDSDGSFFLYSKLTVDKSRWQQGNVFSCSVLHEALHSHYTQKSLSLSPGK

SEQ ID NO: 174 - protein, 107 aa, Artificial Sequence [sequence omitted]

SEQ ID NO: 175 - protein, 330 aa, Artificial Sequence
  SARS-CoV-2 CH1-CH3 G1m17; IgG1*01 LS GAALIE
ASTKGPSVFPLAPSSKSTSGGTAALGCLVKDYFPEPVTVSWNSGALTSGVHTFPAVLQSSGLYSLSSVVTVPSSSLGTQTYICNVNHKPSNTKVDKKVEPKSCDKTHTCPPCPAPELLAGPSVFLFPPKPKDTLMISRTPEVTCVVVDVSHEDPEVKFNWYVDGVEVHNAKTKPREEQYNSTYRVVSVLTVLHQDWLNGKEYKCKVSNKALPLPEEKTISKAKGQPREPQVYTLPPSRDELTKNQVSLTCLVKGFYPSDIAVEWESNGQPENNYKTTPPVLDSDGSFFLYSKLTVDKSRWQQGNVFSCSVLHEALHSHYTQKSLSLSPGK

SEQ ID NO: 176 - protein, 123 aa, Artificial Sequence
  SARS-CoV-2 S300-v2.10 mAb VH
QVQLVQSGAEVKKPGASVKVSCKASGYTFTDYYIHWVRQAPGQGPEWLGFVNAYSGATRYAQKYQGRVTMTRDTSISTAYMQLSRLRPDDTAVYYCARDRPSHEFAMYFFDNWGQGTLVTVSS

SEQ ID NO: 177 - protein, 123 aa, Artificial Sequence
  SARS-CoV-2 S300-v2.11 mAb VH
QVQLVQSGAEVKKPGASVKVSCKASGYTFTDYYIHWVRQAPGQGPEWLGFVQGYSGATRYAQKYQGRVTMTRDTSISTAYMQLSRLRPDDTAVYYCARDRPSHEFAMYFFDNWGQGTLVTVSS

SEQ ID NO: 178 - protein, 124 aa, Artificial Sequence
  SARS-CoV-2 S315-v1 mAb VH
EVQLVESGGGLVQPGGSLRLSCAASGFTFSNYWMTWVRQAPGKGLEWVANIKQDGSEKYYVDSVKGRFTISRDNAKNSLYLQMNSLRAEDTAVYYCARDLWWNDQAHYYGMDVWGQGTTVTVSS

SEQ ID NO: 179 - protein, 8 aa, Artificial Sequence
  SARS-CoV-2 S315-v1 mAb CDRH1
GFTFSNYW

SEQ ID NO: 180 - protein, 8 aa, Artificial Sequence
  SARS-CoV-2 S315-v1 mAb CDRH2
IKQDGSEK

SEQ ID NO: 181 - protein, 17 aa, Artificial Sequence
  SARS-CoV-2 S315-v1 mAb CDRH3
ARDLWWNDQAHYYGMDV

SEQ ID NO: 182 - protein, 106 aa, Artificial Sequence
  SARS-CoV-2 S315-v1 mAb VL
SYELTQPPSVSVSPGQTARITCSGDAFPNQYAYWYQQKPGQAPVMLIYKDSERPSGIPERFFGSSSGTTVTLTIRGVQAEDEADYYCQSADSSGTVFGGGTKLTVL

SEQ ID NO: 183 - protein, 6 aa, Artificial Sequence
  SARS-CoV-2 S315-v1 mAb CDRL1
AFPNQY

SEQ ID NO: 184 - protein, 3 aa, Artificial Sequence
  SARS-CoV-2 S315-v1 mAb CDRL2
KDS

SEQ ID NO: 185 - protein, 9 aa, Artificial Sequence
  SARS-CoV-2 S315-v1 mAb CDRL3
QSADSSGTV

SEQ ID NO: 186 - DNA, 373 bp, Artificial Sequence
  SARS-CoV-2 S315-v1 mAb VH
gaggtgcagctggtggagtctgggggaggcttggtccagcctggggggtccctgagactctcctgtgcagcctctggattcacctttagtaattattggatgacctgggtccgccaggctccagggaaggggctggagtgggtggccaacataaagcaagatggaagtgagaaatactatgtggactctgtgaagggccgattcaccatctccagagacaacgccaagaactcactgtatctgcaaatgaacagcctgagagccgaggacacggctgtgtattactgtgcgagagatctttggtggaacgaccaggctcactactacggtatggacgtctggggccaagggaccacggtcaccgtctcctcag

SEQ ID NO: 187 - DNA, 319 bp, Artificial Sequence
  SARS-CoV-2 S315-v1 mAb VL
tcctatgagctgacacagccaccctcggtgtcagtgtccccaggacagacggccaggatcacctgctctggagatgcattcccaaaccaatatgcttattggtaccagcagaagccaggccaggcccctgtgatgctgatctataaagacagtgagaggccctcagggatccctgagcgattctttggctccagctcagggacaacagtcacgttgaccatcagaggagtccaggcagaagacgaggctgactattactgtcaatcagcagacagcagtggtaccgtgttcggcggagggaccaagctgaccgtcctag

SEQ ID NO: 188 - DNA, 372 bp, Artificial Sequence
  SARS-CoV-2 S315-v1 mAb VH (nt - codon optimized)
gaagtgcagcttgtcgagagcggcggaggcctcgttcagccaggtgggagtctccgtctttcatgcgccgcttcaggatttacgttctccaactactggatgacatgggtgaggcaggcacctgggaaggggctggagtgggtggctaacatcaagcaggacggatctgaaaaatattatgtagattctgtgaaggggcggtttaccatctcaagggataatgccaaaaactctttgtatttacagatgaactctcttcgagccgaggacaccgccgtttactactgtgcccgagatctatggtggaatgaccaggctcactattatggaatggacgtgtggggccagggtactaccgttaccgtctcctca

SEQ ID NO: 189 - DNA, 318 bp, Artificial Sequence
  SARS-CoV-2 S315-v1 mAb VL (nt- codon optimized)
tcttacgagctcacccagccaccctcagtgtcagtgagccctggccaaacagctcgcatcacctgttcaggtgacgcctttccaaatcagtacgcctactggtatcagcagaaacccggccaggcacccgttatgctcatctacaaagattctgagcggccatccggtatccccgaacgctttttcggaagctccagtgggactacagttacacttactatccggggagtgcaagctgaagatgaggccgactattattgccagagcgcagactcctcaggcacagtgtttgggggcgggactaaactaactgtgctg

SEQ ID NO: 190 - protein, 106 aa, Artificial Sequence
  SARS-CoV-2 S315-v2 mAb VL
SYELTQPPSVSVSPGQTARITCSGDAFPNQYAYWYQQKPGQAPVMLIYKDSERPSGIPERFFGSSSGTTVTLTISGVQAEDEADYYCQSADSSGTVFGGGTKLTVL

SEQ ID NO: 191 - DNA, 319 bp, Artificial Sequence
  SARS-CoV-2 S315-v2 mAb VL
tcctatgagctgacacagccaccctcggtgtcagtgtccccaggacagacggccaggatcacctgctctggagatgcattcccaaaccaatatgcttattggtaccagcagaagccaggccaggcccctgtgatgctgatctataaagacagtgagaggccctcagggatccctgagcgattctttggctccagctcagggacaacagtcacgttgaccatcagtggagtccaggcagaagacgaggctgactattactgtcaatcagcagacagcagtggtaccgtgttcggcggagggaccaagctgaccgtcctag

SEQ ID NO: 192 - DNA, 318 bp, Artificial Sequence
  SARS-CoV-2 S315-v2 mAb VL (nt - codon optimized)
tcctacgagctcacccagcccccctcagtctctgtgtctcctggacagacagccagaatcacctgctcgggagatgcttttcccaaccaatacgcctactggtaccaacagaaaccaggtcaggcgcctgtcatgctgatttataaagactcagagcggccttcaggaattcccgaaagattcttcgggagttcaagcggaactaccgtgaccttaaccataagcggggtgcaggccgaagatgaagcagactattattgccagagtgccgatagtagtggcacagtctttgggggggggacaaagctgacagtactc

SEQ ID NO: 193 - protein, 106 aa, Artificial Sequence
  SARS-CoV-2 mAb CL IgLC*01
GQPKAAPSVTLFPPSSEELQANKATLVCLISDFYPGAVTVAWKADSSPVKAGVETTTPSKQSNNKYAASSYLSLTPEQWKSHRSYSCQVTHEGSTVEKTVAPTECS

SEQ ID NO: 194 - protein, 124 aa, Artificial Sequence
  SARS-CoV-2 S315-v3 mAb VH
EVQLVESGGGLVQPGGSLRLSCAASGFTFSNYFMTWVRQAPGKGLEWVANIKQDGSEKYYVDSVKGRFTISRDNAKNSLYLQMNSLRAEDTAVYYCARDLWWNDQAHYYGMDVWGQGTTVTVSS

SEQ ID NO: 195 - protein, 8 aa, Artificial Sequence
  SARS-CoV-2 S315-v3 mAb CDRH1
GFTFSNYF

SEQ ID NO: 196 - protein, 124 aa, Artificial Sequence
  SARS-CoV-2 S315-v4 mAb VH
EVQLVESGGGLVQPGGSLRLSCAASGFTFSNYWMTWVRQAPGKGLEWVANIKQDASEKYYVDSVKGRFTISRDNAKNSLYLQMNSLRAEDTAVYYCARDLWWNDQAHYYGMDVWGQGTTVTVSS

SEQ ID NO: 197 - protein, 8 aa, Artificial Sequence
  SARS-CoV-2 S315-v4 mAb CDRH2
IKQDASEK

SEQ ID NO: 198 - protein, 124 aa, Artificial Sequence
  SARS-CoV-2 S315-v5 mAb VH
EVQLVESGGGLVQPGGSLRLSCAASGFTFSNYWMTWVRQAPGKGLEWVANIKQEGSEKYYVDSVKGRFTISRDNAKNSLYLQMNSLRAEDTAVYYCARDLWWNDQAHYYGMDVWGQGTTVTVSS

SEQ ID NO: 199 - protein, 8 aa, Artificial Sequence
  SARS-CoV-2 S315-v5 mAb CDRH2
IKQEGSEK

SEQ ID NO: 200 - protein, 124 aa, Artificial Sequence
  SARS-CoV-2 S315-v6 mAb VH
EVQLVESGGGLVQPGGSLRLSCAASGFTFSNYWMTWVRQAPGKGLEWVANIKQDGSEKYYVDSVKGRFTISRDNAKNSLYLQMNSLRAEDTAVYYCARDLFWNDQAHYYGMDVWGQGTTVTVSS

SEQ ID NO: 201 - protein, 17 aa, Artificial Sequence
  SARS-CoV-2 S315-v6 mAb CDRH3
ARDLFWNDQAHYYGMDV

SEQ ID NO: 202 - protein, 124 aa, Artificial Sequence
  SARS-CoV-2 S315-v7 mAb VH
EVQLVESGGGLVQPGGSLRLSCAASGFTFSNYWMTWVRQAPGKGLEWVANIKQDGSEKYYVDSVKGRFTISRDNAKNSLYLQMNSLRAEDTAVYYCARDLWFNDQAHYYGMDVWGQGTTVTVSS

SEQ ID NO: 203 - protein, 17 aa, Artificial Sequence
  SARS-CoV-2 S315-v7 mAb CDRH3
ARDLWFNDQAHYYGMDV

SEQ ID NO: 204 - protein, 230 aa, Artificial Sequence
  SARS-CoV-2 Heavy Chain IgHG1*01 Fd
QVQLVQSGAEVKKPGASVKVSCKASGYPFTSYGISWVRQAPGQGLEWMGWISTYNGNTNYAQKFQGRVTMTTDTSTTTGYMELRRLRSDDTAVYYCARDYTRGAWFGESLIGGFDNWGQGTLVTVSSASTKGPSVFPLAPSSKSTSGGTAALGCLVKDYFPEPVTVSWNSGALTSGVHTFPAVLQSSGLYSLSSVVTVPSSSLGTQTYICNVNHKPSNTKVDKRVEPKSC

SEQ ID NO: 205 - protein, 214 aa, Artificial Sequence
  SARS-CoV-2 Light Chain IgKC*01
EIVLTQSPGTLSLSPGERATLSCRASQTVSSTSLAWYQQKPGQAPRLLIYGASSRATGIPDRFSGSGSGTDFTLTISRLEPEDFAVYYCQQHDTSLTFGGGTKVEIKRTVAAPSVFIFPPSDEQLKSGTASVVCLLNNFYPREAKVQWKVDNALQSGNSQESVTEQDSKDSTYSLSSTLTLSKADYEKHKVYACEVTHQGLSSPVTKSFNRGEC

SEQ ID NO: 206 - protein, 18 aa, Artificial Sequence
  Linker
GSTSGSGKPGSGEGSTKG

SEQ ID NO: 207 - protein, 10 aa, Artificial Sequence
  Linker
GSGKPGSGEG

SEQ ID NO: 208 - protein, 8 aa, Artificial Sequence
  Linker
GKPGSGEG

SEQ ID NO: 209 - protein, 8 aa, Artificial Sequence
  Linker
SGKPGSGE

SEQ ID NO: 210 - protein, 6 aa, Artificial Sequence
  Linker
  VARIANT 1: Xaa = positively charged amino acid and Z is glycine or a negatively charged amino acid
  VARIANT (3)...(5): Xaa = Gly or Ser
XPXXXZ

SEQ ID NO: 211 - protein, 121 aa, Artificial Sequence
  Linker
  VARIANT (2)...(10): any one or all of amino acids 2-10 can either be present or absent
  VARIANT (12)...(121): any one or all of amino acids 12-121 can either be present or absent
GGGGGGGGGGSGGGGGGGGGGSGGGGGGGGGGSGGGGGGGGGGSGGGGGGGGGGSGGGGGGGGGGSGGGGGGGGGGSGGGGGGGGGGSGGGGGGGGGGSGGGGGGGGGGSGGGGGGGGGGS

SEQ ID NO: 212 - protein, 15 aa, Artificial Sequence
  Linker
GGGGSGGGGSGGGGS

SEQ ID NO: 213 - protein, 50 aa, Artificial Sequence
  Linker
GGGGSGGGGSGGGGSGGGGSGGGGSGGGGSGGGGSGGGGSGGGGSGGGGS

SEQ ID NO: 214 - protein, 18 aa, Artificial Sequence
  Linker
GSTSGGGSGGGSGGGGSS

SEQ ID NO: 215 - protein, 14 aa, Artificial Sequence
  Linker
EGKSSGSGSESKVD

SEQ ID NO: 216 - protein, 18 aa, Artificial Sequence
  Linker
KESGSVSSEQLAQFRSLD

SEQ ID NO: 217 - protein, 5 aa, Artificial Sequence
  Linker
GGGGS

SEQ ID NO: 218 - protein, 494 aa, Artificial Sequence
  SARS-CoV-2 Synthetic sequence S309-scFab (H-L)
QVQLVQSGAEVKKPGASVKVSCKASGYPFTSYGISWVRQAPGQGLEWMGWISTYNGNTNYAQKFQGRVTMTTDTSTTTGYMELRRLRSDDTAVYYCARDYTRGAWFGESLIGGFDNWGQGTLVTVSSASTKGPSVFPLAPSSKSTSGGTAALGCLVKDYFPEPVTVSWNSGALTSGVHTFPAVLQSSGLYSLSSVVTVPSSSLGTQTYICNVNHKPSNTKVDKRVEPKSCGGGGSGGGGSGGGGSGGGGSGGGGSGGGGSGGGGSGGGGSGGGGSGGGGSEIVLTQSPGTLSLSPGERATLSCRASQTVSSTSLAWYQQKPGQAPRLLIYGASSRATGIPDRFSGSGSGTDFTLTISRLEPEDFAVYYCQQHDTSLTFGGGTKVEIKRTVAAPSVFIFPPSDEQLKSGTASVVCLLNNFYPREAKVQWKVDNALQSGNSQESVTEQDSKDSTYSLSSTLTLSKADYEKHKVYACEVTHQGLSSPVTKSFNRGEC

SEQ ID NO: 219 - protein, 494 aa, Artificial Sequence
  SARS-CoV-2 S309-scFab (L-H)
EIVLTQSPGTLSLSPGERATLSCRASQTVSSTSLAWYQQKPGQAPRLLIYGASSRATGIPDRFSGSGSGTDFTLTISRLEPEDFAVYYCQQHDTSLTFGGGTKVEIKRTVAAPSVFIFPPSDEQLKSGTASVVCLLNNFYPREAKVQWKVDNALQSGNSQESVTEQDSKDSTYSLSSTLTLSKADYEKHKVYACEVTHQGLSSPVTKSFNRGECGGGGSGGGGSGGGGSGGGGSGGGGSGGGGSGGGGSGGGGSGGGGSGGGGSQVQLVQSGAEVKKPGASVKVSCKASGYPFTSYGISWVRQAPGQGLEWMGWISTYNGNTNYAQKFQGRVTMTTDTSTTTGYMELRRLRSDDTAVYYCARDYTRGAWFGESLIGGFDNWGQGTLVTVSSASTKGPSVFPLAPSSKSTSGGTAALGCLVKDYFPEPVTVSWNSGALTSGVHTFPAVLQSSGLYSLSSVVTVPSSSLGTQTYICNVNHKPSNTKVDKRVEPKSC

SEQ ID NO: 220 - protein, 249 aa, Artificial Sequence
  SARS-CoV-2 S309-scFv (VH-VL)
QVQLVQSGAEVKKPGASVKVSCKASGYPFTSYGISWVRQAPGQGLEWMGWISTYNGNTNYAQKFQGRVTMTTDTSTTTGYMELRRLRSDDTAVYYCARDYTRGAWFGESLIGGFDNWGQGTLVTVSSGGGGSGGGGSGGGGSEIVLTQSPGTLSLSPGERATLSCRASQTVSSTSLAWYQQKPGQAPRLLIYGASSRATGIPDRFSGSGSGTDFTLTISRLEPEDFAVYYCQQHDTSLTFGGGTKVEIK

SEQ ID NO: 221 - protein, 249 aa, Artificial Sequence
  SARS-CoV-2 S309-scFv (VL-VH)
EIVLTQSPGTLSLSPGERATLSCRASQTVSSTSLAWYQQKPGQAPRLLIYGASSRATGIPDRFSGSGSGTDFTLTISRLEPEDFAVYYCQQHDTSLTFGGGTKVEIKGGGGSGGGGSGGGGSQVQLVQSGAEVKKPGASVKVSCKASGYPFTSYGISWVRQAPGQGLEWMGWISTYNGNTNYAQKFQGRVTMTTDTSTTTGYMELRRLRSDDTAVYYCARDYTRGAWFGESLIGGFDNWGQGTLVTVSS

SEQ ID NO: 222 - protein, 518 aa, Artificial Sequence
  SARS-CoV-2 S309-scFv (VH-VL)-(VH-VL)
QVQLVQSGAEVKKPGASVKVSCKASGYPFTSYGISWVRQAPGQGLEWMGWISTYNGNTNYAQKFQGRVTMTTDTSTTTGYMELRRLRSDDTAVYYCARDYTRGAWFGESLIGGFDNWGQGTLVTVSSGGGGSGGGGSGGGGSEIVLTQSPGTLSLSPGERATLSCRASQTVSSTSLAWYQQKPGQAPRLLIYGASSRATGIPDRFSGSGSGTDFTLTISRLEPEDFAVYYCQQHDTSLTFGGGTKVEIKGGGGSGGGGSGGGGSGGGGSQVQLVQSGAEVKKPGASVKVSCKASGYPFTSYGISWVRQAPGQGLEWMGWISTYNGNTNYAQKFQGRVTMTTDTSTTTGYMELRRLRSDDTAVYYCARDYTRGAWFGESLIGGFDNWGQGTLVTVSSGGGGSGGGGSGGGGSEIVLTQSPGTLSLSPGERATLSCRASQTVSSTSLAWYQQKPGQAPRLLIYGASSRATGIPDRFSGSGSGTDFTLTISRLEPEDFAVYYCQQHDTSLTFGGGTKVEIK

SEQ ID NO: 223 - protein, 518 aa, Artificial Sequence
  SARS-CoV-2 S309-scFv-(VH-VL)-(VL-VH)
QVQLVQSGAEVKKPGASVKVSCKASGYPFTSYGISWVRQAPGQGLEWMGWISTYNGNTNYAQKFQGRVTMTTDTSTTTGYMELRRLRSDDTAVYYCARDYTRGAWFGESLIGGFDNWGQGTLVTVSSGGGGSGGGGSGGGGSEIVLTQSPGTLSLSPGERATLSCRASQTVSSTSLAWYQQKPGQAPRLLIYGASSRATGIPDRFSGSGSGTDFTLTISRLEPEDFAVYYCQQHDTSLTFGGGTKVEIKGGGGSGGGGSGGGGSGGGGSEIVLTQSPGTLSLSPGERATLSCRASQTVSSTSLAWYQQKPGQAPRLLIYGASSRATGIPDRFSGSGSGTDFTLTISRLEPEDFAVYYCQQHDTSLTFGGGTKVEIKGGGGSGGGGSGGGGSQVQLVQSGAEVKKPGASVKVSCKASGYPFTSYGISWVRQAPGQGLEWMGWISTYNGNTNYAQKFQGRVTMTTDTSTTTGYMELRRLRSDDTAVYYCARDYTRGAWFGESLIGGFDNWGQGTLVTVSS

SEQ ID NO: 224 - protein, 518 aa, Artificial Sequence
  SARS-CoV-2 S309-scFv-(VL-VH)-(VH-VL)
EIVLTQSPGTLSLSPGERATLSCRASQTVSSTSLAWYQQKPGQAPRLLIYGASSRATGIPDRFSGSGSGTDFTLTISRLEPEDFAVYYCQQHDTSLTFGGGTKVEIKGGGGSGGGGSGGGGSQVQLVQSGAEVKKPGASVKVSCKASGYPFTSYGISWVRQAPGQGLEWMGWISTYNGNTNYAQKFQGRVTMTTDTSTTTGYMELRRLRSDDTAVYYCARDYTRGAWFGESLIGGFDNWGQGTLVTVSSGGGGSGGGGSGGGGSGGGGSQVQLVQSGAEVKKPGASVKVSCKASGYPFTSYGISWVRQAPGQGLEWMGWISTYNGNTNYAQKFQGRVTMTTDTSTTTGYMELRRLRSDDTAVYYCARDYTRGAWFGESLIGGFDNWGQGTLVTVSSGGGGSGGGGSGGGGSEIVLTQSPGTLSLSPGERATLSCRASQTVSSTSLAWYQQKPGQAPRLLIYGASSRATGIPDRFSGSGSGTDFTLTISRLEPEDFAVYYCQQHDTSLTFGGGTKVEIK

SEQ ID NO: 225 - protein, 518 aa, Artificial Sequence
  Synthetic sequence SARS-CoV-2 S309-scFv-(VL-VH)-(VL-VH)
EIVLTQSPGTLSLSPGERATLSCRASQTVSSTSLAWYQQKPGQAPRLLIYGASSRATGIPDRFSGSGSGTDFTLTISRLEPEDFAVYYCQQHDTSLTFGGGTKVEIKGGGGSGGGGSGGGGSQVQLVQSGAEVKKPGASVKVSCKASGYPFTSYGISWVRQAPGQGLEWMGWISTYNGNTNYAQKFQGRVTMTTDTSTTTGYMELRRLRSDDTAVYYCARDYTRGAWFGESLIGGFDNWGQGTLVTVSSGGGGSGGGGSGGGGSGGGGSEIVLTQSPGTLSLSPGERATLSCRASQTVSSTSLAWYQQKPGQAPRLLIYGASSRATGIPDRFSGSGSGTDFTLTISRLEPEDFAVYYCQQHDTSLTFGGGTKVEIKGGGGSGGGGSGGGGSQVQLVQSGAEVKKPGASVKVSCKASGYPFTSYGISWVRQAPGQGLEWMGWISTYNGNTNYAQKFQGRVTMTTDTSTTTGYMELRRLRSDDTAVYYCARDYTRGAWFGESLIGGFDNWGQGTLVTVSS

SEQ ID NO: 226 - protein, 494 aa, Artificial Sequence
  Synthetic sequence SARS-CoV-2 S309-scFab-(H-L) v1.1
QVQLVQSGAEVKKPGASVKVSCKASGYPFTSYGISWVRQAPGQGLEWMGWISTYQGNTNYAQKFQGRVTMTTDTSTTTGYMELRRLRSDDTAVYYCARDYTRGAWFGESLIGGFDNWGQGTLVTVSSASTKGPSVFPLAPSSKSTSGGTAALGCLVKDYFPEPVTVSWNSGALTSGVHTFPAVLQSSGLYSLSSVVTVPSSSLGTQTYICNVNHKPSNTKVDKRVEPKSCGGGGSGGGGSGGGGSGGGGSGGGGSGGGGSGGGGSGGGGSGGGGSGGGGSEIVLTQSPGTLSLSPGERATLSCRASQTVSSTSLAWYQQKPGQAPRLLIYGASSRATGIPDRFSGSGSGTDFTLTISRLEPEDFAVYYCQQHDTSLTFGGGTKVEIKRTVAAPSVFIFPPSDEQLKSGTASVVCLLNNFYPREAKVQWKVDNALQSGNSQESVTEQDSKDSTYSLSSTLTLSKADYEKHKVYACEVTHQGLSSPVTKSFNRGEC

SEQ ID NO: 227 - protein, 494 aa, Artificial Sequence
  Synthetic sequence SARS-CoV-2 S309-scFab-(L-H) v1.1
EIVLTQSPGTLSLSPGERATLSCRASQTVSSTSLAWYQQKPGQAPRLLIYGASSRATGIPDRFSGSGSGTDFTLTISRLEPEDFAVYYCQQHDTSLTFGGGTKVEIKRTVAAPSVFIFPPSDEQLKSGTASVVCLLNNFYPREAKVQWKVDNALQSGNSQESVTEQDSKDSTYSLSSTLTLSKADYEKHKVYACEVTHQGLSSPVTKSFNRGECGGGGSGGGGSGGGGSGGGGSGGGGSGGGGSGGGGSGGGGSGGGGSGGGGSQVQLVQSGAEVKKPGASVKVSCKASGYPFTSYGISWVRQAPGQGLEWMGWISTYQGNTNYAQKFQGRVTMTTDTSTTTGYMELRRLRSDDTAVYYCARDYTRGAWFGESLIGGFDNWGQGTLVTVSSASTKGPSVFPLAPSSKSTSGGTAALGCLVKDYFPEPVTVSWNSGALTSGVHTFPAVLQSSGLYSLSSVVTVPSSSLGTQTYICNVNHKPSNTKVDKRVEPKSC

SEQ ID NO: 228 - protein, 249 aa, Artificial Sequence
  Synthetic sequence SARS-CoV-2 S309-scFv-(VH-VL) v1.1
QVQLVQSGAEVKKPGASVKVSCKASGYPFTSYGISWVRQAPGQGLEWMGWISTYQGNTNYAQKFQGRVTMTTDTSTTTGYMELRRLRSDDTAVYYCARDYTRGAWFGESLIGGFDNWGQGTLVTVSSGGGGSGGGGSGGGGSEIVLTQSPGTLSLSPGERATLSCRASQTVSSTSLAWYQQKPGQAPRLLIYGASSRATGIPDRFSGSGSGTDFTLTISRLEPEDFAVYYCQQHDTSLTFGGGTKVEIK

SEQ ID NO: 229 - protein, 249 aa, Artificial Sequence
  Synthetic sequence SARS-CoV-2 S309-scFv-(VL-VH) v1.1
EIVLTQSPGTLSLSPGERATLSCRASQTVSSTSLAWYQQKPGQAPRLLIYGASSRATGIPDRFSGSGSGTDFTLTISRLEPEDFAVYYCQQHDTSLTFGGGTKVEIKGGGGSGGGGSGGGGSQVQLVQSGAEVKKPGASVKVSCKASGYPFTSYGISWVRQAPGQGLEWMGWISTYQGNTNYAQKFQGRVTMTTDTSTTTGYMELRRLRSDDTAVYYCARDYTRGAWFGESLIGGFDNWGQGTLVTVSS

SEQ ID NO: 230 - protein, 518 aa, Artificial Sequence
  Synthetic sequence SARS-CoV-2 S309-scFv-(VH-VL)-(VH-VL) v1.1
QVQLVQSGAEVKKPGASVKVSCKASGYPFTSYGISWVRQAPGQGLEWMGWISTYQGNTNYAQKFQGRVTMTTDTSTTTGYMELRRLRSDDTAVYYCARDYTRGAWFGESLIGGFDNWGQGTLVTVSSGGGGSGGGGSGGGGSEIVLTQSPGTLSLSPGERATLSCRASQTVSSTSLAWYQQKPGQAPRLLIYGASSRATGIPDRFSGSGSGTDFTLTISRLEPEDFAVYYCQQHDTSLTFGGGTKVEIKGGGGSGGGGSGGGGSGGGGSQVQLVQSGAEVKKPGASVKVSCKASGYPFTSYGISWVRQAPGQGLEWMGWISTYQGNTNYAQKFQGRVTMTTDTSTTTGYMELRRLRSDDTAVYYCARDYTRGAWFGESLIGGFDNWGQGTLVTVSSGGGGSGGGGSGGGGSEIVLTQSPGTLSLSPGERATLSCRASQTVSSTSLAWYQQKPGQAPRLLIYGASSRATGIPDRFSGSGSGTDFTLTISRLEPEDFAVYYCQQHDTSLTFGGGTKVEIK

SEQ ID NO: 231 - protein, 518 aa, Artificial Sequence
  Synthetic sequence SARS-CoV-2 S309-scFv-(VH-VL)-(VL-VH) v1.1
QVQLVQSGAEVKKPGASVKVSCKASGYPFTSYGISWVRQAPGQGLEWMGWISTYQGNTNYAQKFQGRVTMTTDTSTTTGYMELRRLRSDDTAVYYCARDYTRGAWFGESLIGGFDNWGQGTLVTVSSGGGGSGGGGSGGGGSEIVLTQSPGTLSLSPGERATLSCRASQTVSSTSLAWYQQKPGQAPRLLIYGASSRATGIPDRFSGSGSGTDFTLTISRLEPEDFAVYYCQQHDTSLTFGGGTKVEIKGGGGSGGGGSGGGGSGGGGSEIVLTQSPGTLSLSPGERATLSCRASQTVSSTSLAWYQQKPGQAPRLLIYGASSRATGIPDRFSGSGSGTDFTLTISRLEPEDFAVYYCQQHDTSLTFGGGTKVEIKGGGGSGGGGSGGGGSQVQLVQSGAEVKKPGASVKVSCKASGYPFTSYGISWVRQAPGQGLEWMGWISTYQGNTNYAQKFQGRVTMTTDTSTTTGYMELRRLRSDDTAVYYCARDYTRGAWFGESLIGGFDNWGQGTLVTVSS

SEQ ID NO: 232 - protein, 518 aa, Artificial Sequence
  Synthetic sequence SARS-CoV-2 S309-scFv-(VH-VL)-(VL-VH) v1.1
EIVLTQSPGTLSLSPGERATLSCRASQTVSSTSLAWYQQKPGQAPRLLIYGASSRATGIPDRFSGSGSGTDFTLTISRLEPEDFAVYYCQQHDTSLTFGGGTKVEIKGGGGSGGGGSGGGGSQVQLVQSGAEVKKPGASVKVSCKASGYPFTSYGISWVRQAPGQGLEWMGWISTYQGNTNYAQKFQGRVTMTTDTSTTTGYMELRRLRSDDTAVYYCARDYTRGAWFGESLIGGFDNWGQGTLVTVSSGGGGSGGGGSGGGGSGGGGSQVQLVQSGAEVKKPGASVKVSCKASGYPFTSYGISWVRQAPGQGLEWMGWISTYQGNTNYAQKFQGRVTMTTDTSTTTGYMELRRLRSDDTAVYYCARDYTRGAWFGESLIGGFDNWGQGTLVTVSSGGGGSGGGGSGGGGSEIVLTQSPGTLSLSPGERATLSCRASQTVSSTSLAWYQQKPGQAPRLLIYGASSRATGIPDRFSGSGSGTDFTLTISRLEPEDFAVYYCQQHDTSLTFGGGTKVEIK

SEQ ID NO: 233 - protein, 518 aa, Artificial Sequence
  Synthetic sequence SARS-CoV-2 S309-scFv-(VL-VH)-(VL-VH) v1.1
EIVLTQSPGTLSLSPGERATLSCRASQTVSSTSLAWYQQKPGQAPRLLIYGASSRATGIPDRFSGSGSGTDFTLTISRLEPEDFAVYYCQQHDTSLTFGGGTKVEIKGGGGSGGGGSGGGGSQVQLVQSGAEVKKPGASVKVSCKASGYPFTSYGISWVRQAPGQGLEWMGWISTYQGNTNYAQKFQGRVTMTTDTSTTTGYMELRRLRSDDTAVYYCARDYTRGAWFGESLIGGFDNWGQGTLVTVSSGGGGSGGGGSGGGGSGGGGSEIVLTQSPGTLSLSPGERATLSCRASQTVSSTSLAWYQQKPGQAPRLLIYGASSRATGIPDRFSGSGSGTDFTLTISRLEPEDFAVYYCQQHDTSLTFGGGTKVEIKGGGGSGGGGSGGGGSQVQLVQSGAEVKKPGASVKVSCKASGYPFTSYGISWVRQAPGQGLEWMGWISTYQGNTNYAQKFQGRVTMTTDTSTTTGYMELRRLRSDDTAVYYCARDYTRGAWFGESLIGGFDNWGQGTLVTVSS

SEQ ID NO: 234 - protein, 114 aa, Artificial Sequence
  Synthetic sequence SARS-CoV-2 S300-v14 mAb VL (VK)
DIVMTQSPDSLAVSLGERATINCKSSQSVLYSSNNKNYLAWYQQKPGQPPKLLISWASTRESGVPDRFSGSGSGTDFTLTISSLQAEDVAVYYCQQYYSAPGITFGQGTRLEIK

SEQ ID NO: 235 - protein, 12 aa, Artificial Sequence
  Synthetic sequence SARS-CoV-2 S300-v14 mAb CDRL1
QSVLYSSNNKNY

SEQ ID NO: 236 - protein, 3 aa, Artificial Sequence
  Synthetic sequence SARS-CoV-2 S300-v14 mAb CDRL2
WAS

SEQ ID NO: 237 - protein, 10 aa, Artificial Sequence
  Synthetic sequence SARS-CoV-2 S300-v14 mAb CDRL3
QQYYSAPGIT

SEQ ID NO: 238 - DNA, 343 bp, Artificial Sequence
  Synthetic sequence SARS-CoV2 S300-v14 mAb VL (VK)
gacatcgtgatgacccagtctccagactcactggctgtgtctctgggcgagagggccaccatcaactgtaagtccagccagagtgttttatacagctccaacaataagaactacttagcttggtaccagcagaaaccaggacagcctcctaagctgctcatttcctgggcttctacccgggaatccggggtccctgaccgattcagtggcagcgggtctgggacagatttcactctcaccatcagcagcctgcaggctgaagatgtggcagtttattactgtcaacaatattatagtgctcccgggatcaccttcggccaggggacacgactggagattaaac

SEQ ID NO: 239 - protein, 129 aa, Artificial Sequence
  Synthetic sequence SARS-CoV2 S307 mAb VH
QVQLQESGPGLVKPSETLSLTCTVSGGSVTSGSYYWSWIRQPPGKGLEWIGYMYYSGSTNYNPSLKSRVTISVDTSKNQFSLKLSSVTAADTAVYYCARAGCTGITCLRYDYYYGLDVWGQGTTVTVSS

SEQ ID NO: 240 - protein, 10 aa, Artificial Sequence
  Synthetic sequence SARS-CoV2 S307 mAb CDRH1
GGSVTSGSYY

SEQ ID NO: 241 - protein, 7 aa, Artificial Sequence
  Synthetic sequence SARS-CoV2 S307 mAb CDRH2
MYYSGST

SEQ ID NO: 242 - protein, 21 aa, Artificial Sequence
  Synthetic sequence SARS-CoV2 S307 mAb CDRH3
ARAGCTGITCLRYDYYYGLDV

SEQ ID NO: 243 - protein, 108 aa, Artificial Sequence
  Synthetic sequence SARS-CoV2 S307 mAb VL(VK)
EIVLTQSPGTLSLSPGKRATLSCRASQSVSSSYLAWYQQRPGQAPRLLIYGASSRAAGIPDRFSGSGSGTDFTLTISRLEPEDFAVYYCQQYGSSSWTFGQGTKVEIK

SEQ ID NO: 244 - protein, 7 aa, Artificial Sequence
  Synthetic sequence SARS-CoV2 S307 mAb CDRL1
QSVSSSY

SEQ ID NO: 245 - protein, 3 aa, Artificial Sequence
  Synthetic sequence SARS-CoV2 S307 mAb CDRL2
GAS

SEQ ID NO: 246 - protein, 9 aa, Artificial Sequence
  Synthetic sequence SARS-CoV2 S307 mAb CDRL3
QQYGSSSWT

SEQ ID NO: 247 - DNA, 387 bp, Artificial Sequence
  Synthetic sequence SARS-CoV2 S307 mAb VH
caggtgcagctgcaggagtcgggcccaggactggtgaagccttcggagaccctgtccctcacctgcactgtctctggtggctccgtcaccagtggtagttactactggagctggatccggcagcccccagggaagggactggagtggattgggtatatgtattacagtgggagcaccaattacaacccctccctcaagagtcgagtcaccatatcagtagacacgtccaagaaccagttctccctgaagctgagctctgtgaccgctgcggacacggccgtgtattactgtgcgagggcaggttgtactggtatcacctgcttacgttacgactactactacggtctggacgtctggggccaagggaccacggtcaccgtctcctca

SEQ ID NO: 248 - DNA, 325 bp, Artificial Sequence
  Synthetic sequence SARS-CoV2 S307 mAb VL(VK)
gaaattgtgttgacgcagtctccaggcaccctgtctttgtctccagggaaaagagccaccctctcctgcagggccagtcagagtgttagcagcagctacttagcctggtaccagcagagacctggccaggctcccaggctcctcatctatggtgcatccagcagggccgctggcatcccagacaggttcagtggcagtgggtctgggacagacttcactctcaccatcagcagactggagcctgaagattttgcagtgtattactgtcagcagtatggtagctcatcgtggacgttcggccaagggaccaaggtggaaatcaaac

SEQ ID NO: 249 - DNA, 381 bp, Artificial Sequence
  Synthetic sequence SARS-CoV-2 S309-v1 mAb VH
caggttcagctggtgcagtctggagctgaggtgaagaagcctggggcctcagtgaaggtctcctgcaaggcttctggttacccctttaccagttatggtatcagctgggtgcgacaggcccctggacaagggcttgagtggatgggatggatcagcacttacaatggtaacacaaattatgcacagaagttccagggcagagtcaccatgaccacagacacatccacgaccacaggctacatggagctgaggaggctgagatctgacgacacggccgtgtattactgtgcgagagattatactcgtggtgcttggttcggggagtcattgatagggggctttgacaactggggccagggaaccctggtcaccgtctcctca

SEQ ID NO: 250 - DNA, 322 bp, Artificial Sequence
  Synthetic sequence SAES-CoV-2 S309-v13 mAb VL(VK)
gaaattgtgttgacgcagtctccaggcaccctgtctttgtctccaggggaaagagccaccctctcctgcagggccagtcagactgttagcagcacctccttagcctggtaccagcagaaacctggccaggctcccaggctcctcatctatggtgcatccagcagggccactggcatcccagacaggttcagcggcagtgggtctgggacagacttcactctcaccatcagcagactggagcctgaagattttgcagtgtattactgtcagcagcatgatacctcactcactttcggcggagggaccaaggtggagatcaaac

SEQ ID NO: 251 - DNA, 767 bp, Artificial Sequence
  Synthetic sequence CMV promoter
gacattgattattgactagttattaatagtaatcaattacggggtcattagttcatagcccatatatggagttccgcgttacataacttacggtaaatggcccgcctggctgaccgcccaacgacccccgcccatgacgtcaataatgacgtatgttcccatagtaacgccaatagggactttccattgacgtcaatgggtggagtatttacggtaaactgcccacttggcagtacatcaagtgtatcatatgccaagtacgccccctattgacgtcaatgacggtaaatggcccgcctggcattatgcccagtacatgaccttatgggactttcctacttggcagtacatctacgtattagtcatcgctattaccatggtgatgcggttttggcagtacatcaatgggcgtggatagcggtttgactcacggggatttccaagtctccaccccattgacgtcaatgggagtttgttttggcaccaaaatcaacgggactttccaaaatgtcgtaacaactccgccccattgacgcaaatgggcggtaggcgtgtacggtgggaggtctatataagcagagctcgtttagtgaaccgtcagatcgcctggagacgccatccacgctgttttgacctccatagaagacaccgggaccgatccagcctccgcggccgggaacggtgcattggaacgcggattccccgtgccaagagtgacgtaagtaccgcctatagagtctataggcccacccccttggcttcgttag

SEQ ID NO: 252 - DNA, 50 bp, Artificial Sequence
  Signal peptide
atgggatggtcatgtatcatcctttttctagtagcaactgcaaccggtgt

SEQ ID NO: 253 - DNA, 135 bp, Artificial Sequence
  Poly-adenylation signal sequence
aacttgtttattgcagcttataatggttacaaataaagcaatagcatcacaaatttcacaaataaagcatttttttcactgcattctagttgtggtttgtccaaactcatcaatgtatcttatcatgtctggatc

SEQ ID NO: 254 - DNA, 323 bp, Artificial Sequence
  Synthetic sequence SARS-CoV-2 Light Chain IgKC*01
gtacggtggctgcaccatctgtcttcatcttcccgccatctgatgagcagttgaaatctggaactgcctctgttgtgtgcctgctgaataacttctatcccagagaggccaaagtacagtggaaggtggataacgccctccaatcgggtaactcccaggagagtgtcacagagcaggacagcaaggacagcacctacagcctcagcagcaccctgacgctgagcaaagcagactacgagaaacacaaagtctacgcctgcgaagtcacccatcagggcctgagctcgcccgtcacaaagagcttcaacaggggagagtgttag

SEQ ID NO: 255 - DNA, 993 bp, Artificial Sequence
  Synthetic sequence SARS-CoV-2 CH1-CH3 G1m17; IgG1*01
gcgtcgaccaagggcccatcggtcttccccctggcaccctcctccaagagcacctctgggggcacagcggccctgggctgcctggtcaaggactacttccccgaacctgtgacggtctcgtggaactcaggcgccctgaccagcggcgtgcacaccttcccggctgtcctacagtcctcaggactctactccctcagcagcgtggtgaccgtgccctccagcagcttgggcacccagacctacatctgcaacgtgaatcacaagcccagcaacaccaaggtggacaagagagttgagcccaaatcttgtgacaaaactcacacatgcccaccgtgcccagcacctgaactcctggggggaccgtcagtcttcctcttccccccaaaacccaaggacaccctcatgatctcccggacccctgaggtcacatgcgtggtggtggacgtgagccacgaagaccctgaggtcaagttcaactggtacgtggacggcgtggaggtgcataatgccaagacaaagccgcgggaggagcagtacaacagcacgtaccgtgtggtcagcgtcctcaccgtcctgcaccaggactggctgaatggcaaggagtacaagtgcaaggtctccaacaaagccctcccagcccccatcgagaaaaccatctccaaagccaaagggcagccccgagaaccacaggtgtacaccctgcccccatcccgggaggagatgaccaagaaccaggtcagcctgacctgcctggtcaaaggcttctatcccagcgacatcgccgtggagtgggagagcaatgggcagccggagaacaactacaagaccacgcctcccgtgctggactccgacggctccttcttcctctatagcaagctcaccgtggacaagagcaggtggcagcaggggaacgtcttctcatgctccgtgatgcatgaggctctgcacaaccactacacgcagaagagcctctccctgtccccgggtaaatga

SEQ ID NO: 256 - protein, 16 aa, Artificial Sequence
  Signal peptide
MGWSCIILFLVATATG

SEQ ID NO: 257 - DNA, 1431 bp, Artificial Sequence
  Synthetic sequence SARS-CoV-2 S309-v1.1 mAb CH1-CH3 G1m17; IgGHG1*01 LS; GAALIE; signal peptide (nt-CO)
atgggctggtcctgtatcatcctgttcctggtcgccacagccaccggagtgcacagccaagtgcagctggtccagagcggcgccgaggtgaagaagcccggcgctagcgtgaaggtgtcctgtaaagccagcggatatccttttaccagctacggcatctcctgggtgcggcaggcccctggccagggcctggaatggatgggctggatcagcacctaccagggaaataccaactacgcccagaagttccagggaagagtgacaatgaccacagatacatctacaaccaccggctacatggaactgaggcggctgagaagcgacgacaccgccgtgtactactgcgccagagattacaccagaggcgcttggttcggcgagagcctgatcggcggcttcgacaactggggccagggaaccctggtgacagtgtctagcgcttctaccaaaggcccttctgtctttcctctggccccttctagcaagtctacaagcggaggcaccgccgccctgggctgcctggtgaaggactacttccccgagcccgtgaccgtgagctggaatagcggcgccctgacaagcggcgtgcacaccttcccagctgtgctgcagagcagcggcctgtatagcctgagcagcgtggtcaccgtgcccagcagcagcctgggaacacagacctacatctgcaacgtgaaccacaagccttctaataccaaggtggataagaaggtggaacctaagagctgcgacaaaacacacacatgccctccatgtcctgctccagagctgctggccggccccagcgtttttctgttcccccccaaacctaaagacaccctgatgatcagcagaacccctgaggtgacctgtgtggtggtggacgtgtcccacgaagatcctgaggtgaagttcaactggtacgtggatggagtggaagtgcacaacgccaagaccaaacctagagaagagcagtacaacagcacatatagagtcgtgtccgtgcttacagtgctgcaccaggactggctgaatggaaaggaatacaagtgcaaggtgtccaacaaggccctgcctctgcctgaggagaagacaatctctaaagccaagggccaacctcgggaacctcaggtgtacacactgccccccagccgggacgagctgaccaagaaccaggtgtccctgacctgcctggtcaagggcttctacccctctgatatcgccgtggaatgggagagcaacggccaacctgagaacaactacaagaccacccctccagtgctggacagcgacggcagcttcttcctgtacagcaagctgaccgttgacaagtccagatggcagcagggcaacgtgttcagctgtagcgtcctgcacgaggccctgcattctcactacacccagaagagcctgtccctcagccctggcaagtga

SEQ ID NO: 258 - DNA, 1374 bp, Artificial Sequence
  Synthetic sequence SARS-CoV-2 S309-v1.1 mAb CH1-CH3 G1m17; IgGHG1*01 LS; GAALIE; (nt-CO)
caagtgcagctggtccagagcggcgccgaggtgaagaagcccggcgctagcgtgaaggtgtcctgtaaagccagcggatatccttttaccagctacggcatctcctgggtgcggcaggcccctggccagggcctggaatggatgggctggatcagcacctaccagggaaataccaactacgcccagaagttccagggaagagtgacaatgaccacagatacatctacaaccaccggctacatggaactgaggcggctgagaagcgacgacaccgccgtgtactactgcgccagagattacaccagaggcgcttggttcggcgagagcctgatcggcggcttcgacaactggggccagggaaccctggtgacagtgtctagcgcttctaccaaaggcccttctgtctttcctctggccccttctagcaagtctacaagcggaggcaccgccgccctgggctgcctggtgaaggactacttccccgagcccgtgaccgtgagctggaatagcggcgccctgacaagcggcgtgcacaccttcccagctgtgctgcagagcagcggcctgtatagcctgagcagcgtggtcaccgtgcccagcagcagcctgggaacacagacctacatctgcaacgtgaaccacaagccttctaataccaaggtggataagaaggtggaacctaagagctgcgacaaaacacacacatgccctccatgtcctgctccagagctgctggccggccccagcgtttttctgttcccccccaaacctaaagacaccctgatgatcagcagaacccctgaggtgacctgtgtggtggtggacgtgtcccacgaagatcctgaggtgaagttcaactggtacgtggatggagtggaagtgcacaacgccaagaccaaacctagagaagagcagtacaacagcacatatagagtcgtgtccgtgcttacagtgctgcaccaggactggctgaatggaaaggaatacaagtgcaaggtgtccaacaaggccctgcctctgcctgaggagaagacaatctctaaagccaagggccaacctcgggaacctcaggtgtacacactgccccccagccgggacgagctgaccaagaaccaggtgtccctgacctgcctggtcaagggcttctacccctctgatatcgccgtggaatgggagagcaacggccaacctgagaacaactacaagaccacccctccagtgctggacagcgacggcagcttcttcctgtacagcaagctgaccgttgacaagtccagatggcagcagggcaacgtgttcagctgtagcgtcctgcacgaggccctgcattctcactacacccagaagagcctgtccctcagccctggcaagtga

SEQ ID NO: 259 - DNA, 1431 bp, Artificial Sequence
  Synthetic sequence SARS-CoV-2 S309-v1.1 mAb CH1-CH3 G1m17; IgGHG1*01 LS; signal peptide (nt-CO)
atgggctggtcctgtatcatcctgttcctggtcgccacagccaccggagtgcacagccaagtgcagctggtccagagcggcgccgaggtgaagaagcccggcgctagcgtgaaggtgtcctgtaaagccagcggatatccttttaccagctacggcatctcctgggtgcggcaggcccctggccagggcctggaatggatgggctggatcagcacctaccagggaaataccaactacgcccagaagttccagggaagagtgacaatgaccacagatacatctacaaccaccggctacatggaactgaggcggctgagaagcgacgacaccgccgtgtactactgcgccagagattacaccagaggcgcttggttcggcgagagcctgatcggcggcttcgacaactggggccagggaaccctggtgacagtgtctagcgcttctaccaaaggcccttctgtctttcctctggccccttctagcaagtctacaagcggaggcaccgccgccctgggctgcctggtgaaggactacttccccgagcccgtgaccgtgagctggaatagcggcgccctgacaagcggcgtgcacaccttcccagctgtgctgcagagcagcggcctgtatagcctgagcagcgtggtcaccgtgcccagcagcagcctgggaacacagacctacatctgcaacgtgaaccacaagccttctaataccaaggtggataagaaggtggaacctaagagctgcgacaaaacacacacatgccctccatgtcctgctccagagctgctgggcggccccagcgtttttctgttcccccccaaacctaaagacaccctgatgatcagcagaacccctgaggtgacctgtgtggtggtggacgtgtcccacgaagatcctgaggtgaagttcaactggtacgtggatggagtggaagtgcacaacgccaagaccaaacctagagaagagcagtacaacagcacatatagagtcgtgtccgtgcttacagtgctgcaccaggactggctgaatggaaaggaatacaagtgcaaggtgtccaacaaggccctgcctgcccctatcgagaagacaatctctaaagccaagggccaacctcgggaacctcaggtgtacacactgccccccagccgggacgagctgaccaagaaccaggtgtccctgacctgcctggtcaagggcttctacccctctgatatcgccgtggaatgggagagcaacggccaacctgagaacaactacaagaccacccctccagtgctggacagcgacggcagcttcttcctgtacagcaagctgaccgttgacaagtccagatggcagcagggcaacgtgttcagctgtagcgtcctgcacgaggccctgcattctcactacacccagaagagcctgtccctcagccctggcaagtga

SEQ ID NO: 260 - DNA, 1374 bp, Artificial Sequence
  Synthetic sequence SARS-CoV-2 S309-v1.1 mAb CH1-CH3 G1m17; IgGHG1*01 LS (nt-CO)
caagtgcagctggtccagagcggcgccgaggtgaagaagcccggcgctagcgtgaaggtgtcctgtaaagccagcggatatccttttaccagctacggcatctcctgggtgcggcaggcccctggccagggcctggaatggatgggctggatcagcacctaccagggaaataccaactacgcccagaagttccagggaagagtgacaatgaccacagatacatctacaaccaccggctacatggaactgaggcggctgagaagcgacgacaccgccgtgtactactgcgccagagattacaccagaggcgcttggttcggcgagagcctgatcggcggcttcgacaactggggccagggaaccctggtgacagtgtctagcgcttctaccaaaggcccttctgtctttcctctggccccttctagcaagtctacaagcggaggcaccgccgccctgggctgcctggtgaaggactacttccccgagcccgtgaccgtgagctggaatagcggcgccctgacaagcggcgtgcacaccttcccagctgtgctgcagagcagcggcctgtatagcctgagcagcgtggtcaccgtgcccagcagcagcctgggaacacagacctacatctgcaacgtgaaccacaagccttctaataccaaggtggataagaaggtggaacctaagagctgcgacaaaacacacacatgccctccatgtcctgctccagagctgctgggcggccccagcgtttttctgttcccccccaaacctaaagacaccctgatgatcagcagaacccctgaggtgacctgtgtggtggtggacgtgtcccacgaagatcctgaggtgaagttcaactggtacgtggatggagtggaagtgcacaacgccaagaccaaacctagagaagagcagtacaacagcacatatagagtcgtgtccgtgcttacagtgctgcaccaggactggctgaatggaaaggaatacaagtgcaaggtgtccaacaaggccctgcctgcccctatcgagaagacaatctctaaagccaagggccaacctcgggaacctcaggtgtacacactgccccccagccgggacgagctgaccaagaaccaggtgtccctgacctgcctggtcaagggcttctacccctctgatatcgccgtggaatgggagagcaacggccaacctgagaacaactacaagaccacccctccagtgctggacagcgacggcagcttcttcctgtacagcaagctgaccgttgacaagtccagatggcagcagggcaacgtgttcagctgtagcgtcctgcacgaggccctgcattctcactacacccagaagagcctgtccctcagccctggcaagtga

SEQ ID NO: 261 - DNA, 701 bp, Artificial Sequence
  Synthetic sequence S309-v13 Light chain k1m3; IgKC*01; signal peptide (nt-CO)
tgggctggtcctgcatcatcctgttcctggtggccacagccaccggcgtgcacagcgagatcgtcctgacacagagccccggcacactgagcctctccccaggcgagcgggctacactgtcttgtagagcttctcagaccgtgtccagcaccagcctggcctggtatcagcagaaacctggccaggcccctagactgctgatctacggcgccagcagcagagccaccggcatccctgatagattcagcggcagcggatctggaaccgacttcaccctgaccatcagccggctggaacccgaggactttgccgtgtactactgccagcaacacgacaccagcctgaccttcggcggcggaacaaaggtggaaatcaagagaaccgtggccgcccctagcgtgttcatcttcccccccagcgacgagcagctgaagagcggtacagcttctgtggtgtgcctgctgaacaacttctacccgcgggaagccaaggtgcagtggaaggtggacaacgccctgcagagcggcaacagccaggagagcgtgacagagcaggacagcaaggacagcacctacagcctgagcagcaccctgaccctgagcaaggccgactacgagaagcacaaggtgtacgcctgtgaagtgacccaccagggcctgtctagccctgtgaccaagtcttttaacagaggcgagtgctga

SEQ ID NO: 262 - DNA, 645 bp, Artificial Sequence
  Synthetic sequence S309-v13 Light chain k1m3; IgKC*01; (nt-CO)
gagatcgtcctgacacagagccccggcacactgagcctctccccaggcgagcgggctacactgtcttgtagagcttctcagaccgtgtccagcaccagcctggcctggtatcagcagaaacctggccaggcccctagactgctgatctacggcgccagcagcagagccaccggcatccctgatagattcagcggcagcggatctggaaccgacttcaccctgaccatcagccggctggaacccgaggactttgccgtgtactactgccagcaacacgacaccagcctgaccttcggcggcggaacaaaggtggaaatcaagagaaccgtggccgcccctagcgtgttcatcttcccccccagcgacgagcagctgaagagcggtacagcttctgtggtgtgcctgctgaacaacttctacccgcgggaagccaaggtgcagtggaaggtggacaacgccctgcagagcggcaacagccaggagagcgtgacagagcaggacagcaaggacagcacctacagcctgagcagcaccctgaccctgagcaaggccgactacgagaagcacaaggtgtacgcctgtgaagtgacccaccagggcctgtctagccctgtgaccaagtcttttaacagaggcgagtgctga

SEQ ID NO: 263 - DNA, 57 bp, Artificial Sequence
  Signal peptide
atgggctggtcctgcatcatcctgttcctggtggccacagccaccggcgtgcacagc

SEQ ID NO: 264 - protein, 19 aa, Artificial Sequence
  Signal peptide
MGWSCIILFLVATATGVHS

SEQ ID NO: 265 - protein, 329 aa, Artificial Sequence
  Synthetic sequence SARS-CoV-2 CH1-CH3 G1m17; IgG1*01 LS no C-term Lys
ASTKGPSVFPLAPSSKSTSGGTAALGCLVKDYFPEPVTVSWNSGALTSGVHTFPAVLQSSGLYSLSSVVTVPSSSLGTQTYICNVNHKPSNTKVDKKVEPKSCDKTHTCPPCPAPELLGGPSVFLFPPKPKDTLMISRTPEVTCVVVDVSHEDPEVKFNWYVDGVEVHNAKTKPREEQYNSTYRVVSVLTVLHQDWLNGKEYKCKVSNKALPAPIEKTISKAKGQPREPQVYTLPPSRDELTKNQVSLTCLVKGFYPSDIAVEWESNGQPENNYKTTPPVLDSDGSFFLYSKLTVDKSRWQQGNVFSCSVLHEALHSHYTQKSLSLSPG

SEQ ID NO: 266 - protein, 329 aa, Artificial Sequence
  Synthetic sequence SARS-CoV-2 CH1-CH3 G1m17; IgG1*01 LS GAALIE no C-term Lys
ASTKGPSVFPLAPSSKSTSGGTAALGCLVKDYFPEPVTVSWNSGALTSGVHTFPAVLQSSGLYSLSSVVTVPSSSLGTQTYICNVNHKPSNTKVDKKVEPKSCDKTHTCPPCPAPELLAGPSVFLFPPKPKDTLMISRTPEVTCVVVDVSHEDPEVKFNWYVDGVEVHNAKTKPREEQYNSTYRVVSVLTVLHQDWLNGKEYKCKVSNKALPLPEEKTISKAKGQPREPQVYTLPPSRDELTKNQVSLTCLVKGFYPSDIAVEWESNGQPENNYKTTPPVLDSDGSFFLYSKLTVDKSRWQQGNVFSCSVLHEALHSHYTQKSLSLSPG

SEQ ID NO: 267 - protein, 127 aa, Artificial Sequence
  SARS-CoV-2 S309 VH consensus sequence
  VARIANT 50: Xaa = W, F, or Y
  VARIANT 55: Xaa = N, Q, L, or T
  VARIANT 56: Xaa = G, S, A, or Q
  VARIANT 105: Xaa = W, F, or Y
QVQLVQSGAEVKKPGASVKVSCKASGYPFTSYGISWVRQAPGQGLEWMGXISTYXXNTNYAQKFQGRVTMTTDTSTTTGYMELRRLRSDDTAVYYCARDYTRGAXFGESLIGGFDNWGQGTLVTVSS